European Patent Application EP 4 361 279 A2, published May 1, 2024. Title: PATHOGEN-RESISTANT ANIMALS HAVING MODIFIED CD163 GENES. Applicant: The Curators of the University of Missouri. The sequence listing filed with the application follows.

SEQUENCE LISTING (121 sequences)

SEQ ID NO: 1 - DNA, 23 bp, Sus scrofa
  source 1..23: mol_type = other DNA
ggaaacccaggctggttggaggg

SEQ ID NO: 2 - DNA, 23 bp, Sus scrofa
  source 1..23: mol_type = other DNA
ggaactacagtgcggcactgtgg

SEQ ID NO: 3 - DNA, 23 bp, Sus scrofa
  source 1..23: mol_type = other DNA
cagtagcaccccgccctgacggg

SEQ ID NO: 4 - DNA, 23 bp, Sus scrofa
  source 1..23: mol_type = other DNA
tgtagccacagcagggacgtcgg

SEQ ID NO: 5 - DNA, 23 bp, Sus scrofa
  source 1..23: mol_type = other DNA
ccagcctcgcccagcgacatggg

SEQ ID NO: 6 - DNA, 23 bp, Sus scrofa
  source 1..23: mol_type = other DNA
ctttcatttatctgaactcaggg

SEQ ID NO: 7 - DNA, 23 bp, Sus scrofa
  source 1..23: mol_type = other DNA
ttatctgaactcagggtccccgg

SEQ ID NO: 8 - DNA, 23 bp, Sus scrofa
  source 1..23: mol_type = other DNA
cagctgcagcatatatttaaggg

SEQ ID NO: 9 - DNA, 23 bp, synthetic construct
  misc_feature 1..23: note = Synthetic oligonucleotide
  source 1..23: mol_type = other DNA
ctcctcgcccttgctcaccatgg

SEQ ID NO: 10 - DNA, 23 bp, synthetic construct
  misc_feature 1..23: note = Synthetic oligonucleotide
  source 1..23: mol_type = other DNA
gaccaggatgggcaccaccccgg

SEQ ID NO: 11 - DNA, 23 bp, synthetic construct
  misc_feature 1..23: note = Synthetic oligonucleotide
  source 1..23: mol_type = other DNA
ctctccctcactctaacctactt

SEQ ID NO: 12 - DNA, 22 bp, synthetic construct
  misc_feature 1..22: note = Synthetic oligonucleotide
  source 1..22: mol_type = other DNA
tatttctctcacatggccagtc

SEQ ID NO: 13 - DNA, 23 bp, synthetic construct
  misc_feature 1..23: note = Synthetic oligonucleotide
  source 1..23: mol_type = other DNA
ctctccctcactctaacctactt

SEQ ID NO: 14 - DNA, 22 bp, synthetic construct
  misc_feature 1..22: note = Synthetic oligonucleotide
  source 1..22: mol_type = other DNA
gactggccatgtgagagaaata

SEQ ID NO: 15 - DNA, 27767 bp, Sus scrofa
  source 1..27767: mol_type = other DNA
atacaagtgccttttacagacaatctgcacaagttatttgttagacatatttgattatagaattaatattaaaaggggttataacaatcaagcattgataatttaattatgtttgcctattttactttagttttttgacataactgtgtaactattgcgatttttttattcctaatgtaattagttcaaaacaaagtgcagaaatttaaaatattcaattcaacaacagtatataagtcaatattccccccttaaatttttacaaatctttagggagtgtttctcaatttctcaatttctttggttgtttcatgtcccatatggaagaaaacatgggtgtgaaagggaagcttactcttttgattacttcccttttctggttgactccacctccattatgaagcctttctgtatttttgtggaagtgaaatgatttttagaattcttagtggttctcttcttcaggagaacatttctaggtaataatacaagaagatttaaatggcataaaaccttggaatggacaaactcagaatggtgctacatgaaaactctggatctgcaggtaaaatcttctcatttattctatatttaccttttaaatagagtgtagcaatattccgacagtcaatcaatctgatttaatagtgattggcatctggagaagaagtaacagggaaaaaggcaataagctttataaggggaacttttatcttccatagactcaaaattgaagacgtgactagaagattgctagatttggcatcagttttgtaaaattgctgaggtgaaattaagtaagggatgaaaattaactaaattgtgttgagtatgaaactagtagttgttagaaaagatagaacatgaaggaatgaatattgattgaaagttgatgacctagaggacatttagactaacacctctgagtgtcaaagtctaatttatgatttacatcgatgcgttaaactcatttaacattcttacttttttcccctcaagcatttaagctgaagtataacatttcacatgaaagcctggattataaatgcacagttcagtgacctatctcagaggagtgactgccatagcattttttttgtctttttgccttcagagccacagcaacgcgggatccgaagccgcgtctgcgacccacaccacagctcacggcaatgccggatctttaacccactgagcgaggccggggatcgaacccgcagtctcatggttcctagtaggattcgttaaccactgcgccacgacgggaactcctaccatagcatttttacttttaagttactgttggtttagagtaagaaggagaaatgagagtgatggagcgtttgctatatttggagacaaggtcctatattggaggttctcaaatataaattttgtcgctttttcctccaatgtattgttcaactactatttagcaggccactgtgccaggtactggtgaaactggtgaacatgatagatgtaattcattccctcatggaactttccatctaacaatgtggatcaggtaggcttggagatgagaatgccagtggttgactatgactctgtggctgaagggagagctactcacttcgtagtttcatcaatgtctttttggttttccaggttttaagccctgctcttgcaattcttttcccttctccaactttcttctaatttctcacccctaggatgcctataaacatgagtattttcaaagctacttcactgaggttatatgatcctggtgtgaatttttcctgcctgacttgccatttagaaggaagtgtttcctggaatttccattgtggcttggtggttaaagaccctgcattgtctctgtgaggatgtgggttcaatctctggcctcattcagtgagtgggttaaggatctggtgtcgctgcaagctgtggctaagatcccacattgccatgtctgtggtgtagactggcacctggagctctgatttgaccacaatcttaggaacttcagatgtggccataaaaaggaaaaaaaagttaggaagggttttctgtcttgtttggaccttcgttaatctcaaacctttggaaccatctctcctccaaaacctcctttgggtaagactgtatgtttgccctctctcttcttttcgcagactttagaagatgttctgcccatttaagttccttcactttggctgtagtcgctgttctcagtgcctgcttggtcactagttctcttggtgagtactttgacaaatttacttgtaaccgagcccaactgtgacaagaaacactgaaaagcaaataattgctcctgaagtctagatagcatctaaaaacatgcttcatggtttcaaggatcatatattgaaaccccagggatcctctagagtcgacctgcagcatgcaggggggggggggggggggggggggggggggggggggggggggggggggggggggggggggggggggggggggggggggggggggggggggggggggggggggggtgcataaggaaagactatctcaacgtcttattcctcagcttacattagatttgaaactctagtcacctaaaatgcaaatctcatttacttaccatcagagatattaatgacctatagaattcagcataaataaagtttcatgtatggatattagcttatggttctagtcactgctaattgaaacctgtgatattgctgtttgttttgactcctatgaaataacattctcccattgtaccatggatgggtccagaaacatttctcaaatcctggcttgaaaaaataaataagtaatctaaagaataataattctctacttgctctttgaatcttgaccaattgctgcatttacctattgttacaggaggaaaagacaaggagctgaggctaacgggtggtgaaaacaagtgctctggaagagtggaggtgaaagtgcaggaggagtggggaactgtgtgtaataatggctgggacatggatgtggtctctgttgtttgtaggcagctgggatgtccaactgctatcaaagccactggatgggctaattttagtgcaggttctggacgcatttggatggatcatgtttcttgtcgagggaatgagtcagctctctgggactgcaaacatgatggatggggaaagcataactgtactcaccaacaggatgctggagtaacctgctcaggtaagacatacacaaataagtcaagcctatacatgaaatgctttgtgggaaaaaatgtatagatgagttaaaaacaaaaaggaaccagttttctataagtcatctagtccatgtataaaattacccaatccattactaaaagaccacttctggtattttacacatgacaaagcccatattaaaaaaaaaaaattcagaagagattctgaatgctataataaatgagcaagtgactagcttcaattttatattaggtcattctaccttctacttctacatgaaaatatcataatgtctaagttaattccttgtcccctttcccaataaagcactgctttcatgcactggcctatgaatcatgaactttttgccctttaactgatgatcaacttaccaaatcaagaaataaatattcttagcactgatccttttttgttgttgttggaggaagaatgttttgcaaagtagaattgcttttttctgtttaacagtgctattcatttcatttacatggtcgttttaatttataaaacatttcataagtttcacctcatatgcccttacaataactcaggaagttatatgttagacctttctgctgacaaatcccagagtcatgtttctgacccagttcagattccttggcttcccatttctctttgctcatgtcattgacctttatgcagccctcttacctcccacctttctattacagaccatctcctccataggactggtgttagaaagtactaatctctacccaggcattgtggtgcaatgtgggcagcacaggctggtatctagaaaaatgctgaagtgaattccagctcagctgctcgttaatactatcgttttaagtaagctgttcaatcctttgaaattcactttctgagcactcagtgatataataaatgtagagctactggtacactgtctggtatgtaataggtgttaccaattaaccttagtttcctcatgggtcactggttctcattacctagacaactcatttctctttcttcctctttctctttctccattctcctcctccttcttcctcttcttcttgtctgttattgttatatcattttgctgagaaagttaagaaataacaactctaacctctacatcgaccacctagagcaaagttaaaaataataataaaccttgccagactcttactataattgttgctgtctatagagttgactgtttaagttaagacatcagtatatatttttaatttttgtgttttttttttcatacttttacatgaggatcctttatataaggatgagttaaacaaacttgatttttgaagtttatacccctgaggctcaactgcataataatagaaagggatccatagcctctcaaggacttaactagtttcatgagttttcagaatctgaatttctgagattctccaccccaattaaagctcaagcctcagaacatatatccttctcttggtaaattctattcttatcacatgcgtaataataaaaaagagagatgttggagacagatttttttcctcacattctgtctctactgttttctaggtgtttgattctgtgttatttaacctcagtttgcttatctgtgaagtagggattatggtaataacatataatgctttatgttgtaaagactaaagaagatagcatatgtaacacatttggaacagggaatgcatattttgattgtgagctcttattattattaccattcagccctaataaaaatcttggtaagtggaaggctttggatttcagaacttttaaaatctaattactttttcaaaaaagaacttcttagggttttttttttttaaccacaaagtgtttctattttttaggtgtcccaaaatttcgttccaaatatctttttctcagatattttagtcctcatagaacacctagggatagtggatagagaaaattttctttattaaaaagctgttctttgctaaaaattgtagcaggtacttttgggaggggggaaaactttgattcagaaactgctaagacatggagtgttttgactaatttttcctcaatttttaatgttttttataccatagggtacttttgcaaactattatgcatacttatatatttttacttttttcctgtcttttaacttccaaattcaacttcagacaattattcatgcactaaactgtttgtagtaagaaagattaaaattaaaaaattaaccattcaacaaatgactggtttgccatttttactactttgttgtatgaacaatttttttttctacaaatgaatactttgagtctgatttatccattcctacataaaagtttttactatatcttagtattggaaggaaacaaaacaaaacacaatgtaaattttaatctataaattttgggggggtaaatatacatagatgaaagtcttaaccattaattagagtcaaaagattaaaattctccaatatgtgaacttaggctgcatccaaaatgaagcatcatttttaaggacagcatcaaaagtgaccagaggaattttactttctttcttttttttttttttgaattttagtttctaaactcacttctgaataaatacaacttctaaattctcgtcttttctctactctagatggatctgatttagagatgaggctggtgaatggaggaaaccggtgcttaggaagaatagaagtcaaatttcaaggaacgtggggaacagtgtgtgatgatcacttcaacataaatcatgcttctgtggtttgtaaacaacttgaatgtggaagtgctgtcagtttctctggttcagctaattttggagaaggttctggaccaatctggtttgatgatcttgtatgcaatggaaatgagtcagctctctggaactgcaaacatgaaggatggggaaagcacaattgcgatcatgctgaggatgctggagtgatttgcttaagtaaggactgacctgggtttgttctgttctccatgagagggcaaaaaaaggggagtaaaagtcttaaaagctcaaactgttaaaaacataatgatgattgcttcttttatcatcttattattatctaatttcaggtcgaaattctagtacctgtgcagttttttaccttaactgaaattaagataaataggatagggaggaaggatgagcagtgacatttaggtccaagtcatgaggttagaaggaaatgttcagagaatagcccattccctcagccctcaaagaaagaaagaaagaaaaagaaaaaaaaaaagaaagcttaactagaaaattttgttctctggatgttttagaggcaaaccatccctttatcattcctacctacaaagccttctcttaatcacattacccaccctttcctactatagtcaggggggggggggggggggggggggggggggggggggggggggggggggggggggggggggggggggggggggggggggggggggggggggggggggggggtgaaaaaagaaccaaacaatttcaacaaaaaaccaaacaattccaacaaaattggtccaataagcaaacctctagataaatttcagtgccctggatgttttgttaggaactcttcctacaatgcgtgctttccattctgaaaagtcctatctacttgcctgatccacttctccttccatcctaaacgattttcagtggtagtatattactgttgtctctgtctctacttatatatcttccccttttcactcactcctctcaggtacagctcttcagtttgcccttattcttgtttccttgtcaatgacttgttttgtgtccctcttacagatggagcagacctgaaactgagagtggtagatggagtcactgaatgttcaggaagattggaagtgaaattccaaggagaatggggaacaatctgtgatgatggctgggatagtgatgatgccgctgtggcatgtaagcaactgggaggtccaactgctgtcactgccattgtcgagttaacgccagtgagggactggacacattggctcacacacatacagccatgacacgatctgctctatggtccgatgattaaaggggggggggggggggggggggggggggggggggggggggggggggggggggggggggggggggggggggggggggggggggggggggggggggggggggagaagagctggtggacatttctggaaaggaaccaaaacccggaagggccttgttcttcaggatttgggatggattggggagggagaaaattgtttctaatatttcttggtgggaattcttttacagttgtgacaaatctttcacatattcttcatttgagtagtttggagggttgtctgactgttttctataataaatgtcccaagtgctatgaggtaccacatttcaaattctaattctacctgaagctccaaaaagacaaaatgttataggtcttttctttatatctaatttgcttatggtttttagccattgacaatttttttttcttaactcttgaaactataaccctatttctaaccaaattcatgttctatactggctcttcaaaaacccaggagatgggaaagccagaatctccagtgtttcagcttctgggaaggagcaagtttttaaaaataccctctgggagctaaattccacatgtatctatggcctaagtgtatgtttattttgcagatggatcagatctggaactgagacttaaaggtggaggcagccactgtgctgggacagtggaggtggaaattcagaaactggtaggaaaagtgtgtgatagaagctggggactgaaagaagctgatgtggtttgcaggcagctgggatgtggatctgcactcaaaacatcatatcaagtttattccaaaaccaaggcaacaaacacatggctgtttgtaagcagctgtaatggaaatgaaacttctctttgggactgcaagaattggcagtggggtggacttagttgtgatcactatgacgaagccaaaattacctgctcaggtaagaatttcaatcaatgtgttaggaaattgcattctactttcttttacatgtagctgtccagttttcccagcaccacttgttgaagagactgtcttttcttcatcatatagtcctacatcctttgtcataaattaattgaccataggtgtgtgggtttatatctgggctctctattctgttcctttgatctatatgtctgtttttatgccagcaccatgctgttttgattactatagctttgtagtatcatctgaagtcaggaaacatgattcctccagctttgttcttctttctcaagattgttttgtctattcagagtttatgttcccatgcagatttaatttttaaatttatttaatttttattttttatttttaatttaaattaatttaaattttttatttcccaacgtacagccaagggggccagggtaacctttacatgtatacattaaaaatttcaggtttttcccccacccatttctttctgttggcaagtaaatttttgaacaaagtttcccaatgctttttaaggggaattcccttggggggggggggggggggggggggggggggggggggggggggggggggggggggggggggggggggggggggggggggggggggggggggggggggggggggggggggggggggagacgaaattgactatattttctttgttgggaatcttttacagttgtgacaaatctttcacatattcttcatttgagtagtttggagggttgtctgactgttttctataataaatgtcccaagtgctatgaggtaccacatttcaaattctaattctacctgaagctccaaaaagacaaaatgttataggtcttttctttatatctaatttgcttatggtttttagccattgacaatttttttttcttaactcttgaaactataaccctatttctaaccaaattcatgttctatactggctcttcaaaaacccaggagatgggaaagccagaatctccagtgtttcagcttctgggaaggagcaagtttttaaaaataccctctgggagctaaattccacatgtatctatggcctaagtgtatgtttattttgcagatggatcagatctggaactgagacttaaaggtggaggcagccactgtgctgggacagtggaggtggaaattcagaaactggtaggaaaagtgtgtgatagaagctggggactgaaagaagctgatgtggtttgcaggcagctgggatgtggatctgcactcaaaacatcatatcaagtttattccaaaaccaaggcaacaaacacatggctgtttgtaagcagctgtaatggaaatgaaacttctctttgggactgcaagaattggcagtggggtggacttagttgtgatcactatgacgaaaccaaaattacctgctcaggtaagaatttcaatcaatgtgttaggaaaattgcattctactttcttttacatgtagctgtccagttttcccagcaccacttgttgaaaaaactgtctttttcttcatcatatagtcctacatcccttggccataaattaattgaccataaggggtgtgggtttaatatccggggctcctcaattcgggtcccttggatcctaaaagccggttttataacccgacacatggcctgtttttgactaaataaaacctttggaaaacaatcccgaaggtcgaggaacatggaatccccccaacaaaggaccttctttccccaaaaatgcggctcagccaactcaaaaagattttatgaatcacaaaccgcacattatcttcctaaaattactattcctatgttttaatttgcaaagtcattccgatatagttggcgcagagtaactcatttagatatccaccccaccagttcctcactcaagtaaggggggggggggggggggggggggggggggggggggggggggggggggggggggggggggggggggggggggggggggggggggggggggggggggggggcccccatgtgagattttgtgtgtcctttaagagtggagtctctatttcccactgctctctggttctccccaaagtaagccctgctggctttcaaaacttctgggagcttgccttcttggtataggactcctgggctagggagtctaatgtttggcttagaccccttactgcttgggaagaatctctgcaactgtaatgaattatcttcctatttgtgggttgctgaggatatggtcttaactgttctgtgttctacccctcctatccatcttgttgtggttccttctttatatctttagttgtagaaaagtttttcttatcaacagttgctctgtaaattgtaacttgggtgtacacctagtaggaggtgagctcagggtcttcctactctgccatcttggccatgtcctctaaacattttggtgtatttcactgcaacctttttaaaaatctcaaaagtgagctgtgattggctagtcttgtggataatctctagcatttgatgctaatcatatttatacaaatactttgttgaaaagtgatgcctttttaactattattaaaaaacgtattgacataactattgctattatactgaaaagaaagaccttagagaaaatagcataagagcaaaaccattaaacatggagacatctagtcatagggtggaaattttatgtggtccatatcccctaaccagtggctttacaccaggcacatcctaactaagatctgctcccaagtgtcttccctgatgctttaaattgtgttacatggaaactatcctttgatgaagaaatgcaaccttttaaaatacaacattgaaacttttgtgctttaattttgcttttcaacattttttctttttaaaagaagaaatttatttgtttttttaaattttaatggccacggcatatggaagttctcaggccagggatagaattcaagccacaggtgcgacccatgccacaactgctgcaacaccagatcctttaacccactgcaccaggccagggattgaagccttgccttactgacaatctgagccacttcagtcagataaagaaatttcttcattaagcagagtattcacatggtttaaacttcaaaatattaaagtgtaaactctttccccaccactgtccccagctcaccaactctacttaccacagacaactgatgtggttagggtatttaaatagtaaatccaagaaaatataaacaaatccgtatatataggtttcaccccattttattatcctaatgttgcatatcatataaactatactgtcccttgggtattcacttagtaaaatattttgatcataatttcctatcagtatttaaagagctttctgaaattatttctgtataacatttcttttctcatcggtaggggggggggggggggggggggggggggggggggggggggggggggggggggggggggggggggggggggggggggggggggggggggggggggggggggaatgggaagaaaaaaccaccatggttaattttttttatccctctacacccgggaaaattacccttggggccacacttttctatagaaaggggattatttaaaagggtctgaaaaagaatttttttttcgaaaggggaaatatttggcctaacttagtcacataagccatgttctctggcaagttaggtaacatacatttttgtcattgggggcaacaaaaacaattttccttttggaccttttgggactccgcattggttagggaaggggaagtatattggaattcggaaaattccttccaaattaaaaaaggtttgttattttcatattaacctatttcatattaattagcatgaattccagcgccattaaaagggaaaacacctggagtggtaagaaaaaagtttttttttctctttttttttttttttttttaatggccacatctgtggcatgtgaagttcccaggctaggggtcgaataggagctacagctgccagcttgcaccacagccacaacaatgccagagccaagcctcatctgcgacctataccacaactcatggcaatgctggttccttaaccccctgagtgaggcctggggtcaaacccacatcctcatggatactaaccggctttgttaccgctgagccatgagggaaactccctttttctcattgaaaataagtcaaatagataagcagcttaaggctgtttgggtgattctgtggtccagtaattatcaaatcctactggacaagaatagagaatgtgcaaatgagggaacgtgttggtgagatcaggctctgcccactgagctatcctctgtcatgggccctgtgctgttctcagagctgtacttcctagggcattgttctcatttcaattctgagttcagtgtggagagtatacgtgtgtgggggctgcacgcttttcacaacccactttctgctgatactgatttagggatccttggattgctttacagttgagtcatcattaactagtgtcacttgccttcaaagtcagcaaaataattgtctccaaactagtaggcttctagtgtatttgctttaatccaatgccatgtgaaagtaacatggtcaaagaataagttatataccttgacctaccctgtgaccaggctcttcctcttaatttattgaccactgccttaaggtcatttgaaaccatgggtttgggaggaaggcaaggcctaaatcccgtctttgttggaaggctcactgtccttgtctttagagcatcatttttttttaaactggggtacagtttatttacagtgttgtgtcaatttctgctgtacagcacagtgacccagtcatacacatacatacattctttttctcatactatcttcaattttattttctgctaagtctgccattttatcatcacctcagtttgaaggacaggatatttagagtttgttttttttttccccccaatcctgcaatttctaaattataagactctcaattagccgtatataacagctgcaggcacaggatgtctccctcacaaaattggtatttttccttccatttcttcttgcagtttggctatttcttgtctgagttcatctctctttttaagtgttaaaaagggcaaggaggattcatgctatgtcaacattatgattttttcttttctatacttgataagagtatacttttcccaaatgtcatccaacttttcagcatcagtttggacatggttttcttttcaaggtggtatttctctaatgtcacttgaataacaagactcgttagttctccaggctacaatatcctagtctgagtatattctgcatgttaattctattcagccacatccataatttaggttttattcctggaacacctcacttttttttttttttttggtctttttatagccataaccatggcatatggaggttcccaggctaggggtctaatctgagctttagccactggcccatgccacagccacagccatgccacatctgagccacatctgtgaccttttccacagctcacagaaacaccagatccctaacccactgagtgaggccaggggtcaaacctgtaacccttccatggttcctagtcagattcgttcctctgtaccacgatgggaattcctaatacctcacttatgataacacattctgaattatttaggattctattatactgcatgtaatagaaatcccaaatagcaaaatttgcaacttaaggcaggttcctgtctttacaaaatcatgttttcctttgctatatgtgcactttgctttcctctgtgaattcccttttttgttatatttctatagcttttggaaacacttttacttatttgggggggcctagatttttaaccctctccttgtttttctagaaatagagtttataattttatttcttcatttacttgatactttcaagagattcccaggaaaaaaattatggaaatactgtctctgtgcctgccaagttcaaactaagaattgtataatctgttttaattcttaagcatttatagatgacaaggctttgtgtctgataggggccagcgaactcagtaaagagggaagatgagaaagataatggcaagaatttatccctgaagtgtagttttgacaaaccagtcacaaagaggtctaagaaattttggtcacaaagttgttttgaatcccaggcattttatttgcaatgattgcatatgttctggaaaggacatctgaacctaagaaatagttcatttgcattgtgttatattttactaaggtctgagaaataatcttgagatgagaatgaactctacttcttcagagtctggaaggaataaattatgaaaatgtattaatgcttctttaaaccatattgtatatttatctattactaaacaaaaagaagtagctctatttatttatttatttatttatttatttatgtcttttgtctctttagggccacacctgtggcatatggaggttcccaggctagaggtccaattggagatgtagcagccagcctatgccagagccaccgcaacacgggatctgagccacgtctgtgacttacaccacagctcacagcaacgcctgatcctcaacccactgagcgaggccagggatcgaacccatgtcctcatggatgctagttgggttcgttaactgctgagccatgatgggaactccaaattaattatttcttatatttgttcttcatatattcatttctatagaaagaaataaatacagattcagttaatgatggcaggtaaaagcttaacttattaatcaaaggagttaatccaggcacaaaaattcaattcatggctctctgttaaaatttaggtataggtttagcaggaagaaaaggttagtagatgcagactattacatttagaatggatggacaatgaagtcctactatacagcacagggaactatatccaatctcttgggatagaatatgatggaagacaaaatcagaacaagagagtatatatatatgtgtgtgtgtgtgtgtgtgtgtgtgtgtgtgtgtgtgtgtgtgtgactgggtcaccctgcggcacagcagaaattggcagaacattgtaaatcaactatactttaataggaaaaatacttttaagggctaaatttccaatattctaaccatgtacacagagtaaatgtcataaggatgccagtctgtgtagagattgatgtgttactagcagattcatgaaataaaggctgaggatgtagtccccaagtcacttctgagtggaagaatttctcctttgtcctggactcaaatattttaggataaaggaaaaaagaagatatttatagaagggacttgttttcaagtacttgacaaaatttcaccattaaagagaaatttgtgggagttcccatcgtggctcagtggaaacaaatccaactaggaaccatgaggttgtgggtttgatccctggcctcactcagtgggttaaggatccggtgttgccgtgagctgtggtgtaggttgcagacacggttctgatcctgcgttgctgtggctgtggctgtggtgtaggccagcagcaaacagctctgattagacccctagcctggaaacctccatatgccacaggtgcagccctaaaaagacaaaaaaagagaaaagacaaaaaaaaaaaaaaaaaaaaaaaaaaaaaaaaaaaaaaaaaaaagaacccccagaggtatttatttgtttttgccttttttcactgactgttctttgtttgtttgtttgagactgatctagaagactagagattacaagaaatatggatttggctcactctaagaaactgctttcattccaaggtttgggtctatccaaaagtggaatagaatcatatgaatactagtttatgagtatttagtgagaggaatttcaagctcaaataatgattcagcaagattaaattaaggagggaattttccttgtggctgagtgggttaaggacccaatgttgtctctgtgaggatgtaggttccatcctgggctttgctcattaggttaaggatctggcattgctgcagctcagacccagtgctgccctggttgtggcttaggccaaagctgcagctccaattcaatctctggcctgggaacctccatgtgctacaaggtgcggccttaaaaggaaaaaaaaaaaattaaatcaaggactcaagagtctttcattatttgtgttgtggaagctatatttgttttaaagtcttagttgtgtttagaaagcaagatgttcttcaactcaaatttgggagggaacttgtttcatacatttttaatggataagtggcaaaattttcatgctgaggtgatctatagtgttgtaatgcagaatatagtcagatcttgaacattttaggaagttggtgagggccaattgtgtatctgtgccatgctgataagaatgtcaagggatcacaagaattcgtgttatttgacagcagtcatctttaaaaggcatttgagaaagtccaatttcaaatgcatttcctttctttaaaagataaattgaagaaaataagtctttatttcccaagtaaattgaattgcctctcagtctgttaaaagaaactcttaccttgatgattgcgctcttaacctggcaaagattgtctttaaaatctgagctccatgtcttctgctttatttctggtgtgcctttgactccagattacagtaaatggaggactgagtatagggctaaaaagtagagagaatggatgcatattatctgtggtctccaatgtgatgaatgaagtaggcaaatactcaaaggaaagagaaagcatgctccaagaattatgggttccagaaggcaaagtcccagaattgtctccagggaaggacagggaggtctagaatcggctaagcccactgtaggcagaaaaaccaagaggcatgaatggcttccctttctcacttttcactctctggcttactcctatcatgaaggaaaatattggaatcatattctccctcaccgaaatgctatttttcagcccacaggaaacccaggctggttggaggggacattccctgctctggtcgtgttgaagtacaacatggagacacgtggggcaccgtctgtgattctgacttctctctggaggcggccagcgtgctgtgcagggaactacagtgcggcactgtggtttccctcctggggggagctcactttggagaaggaagtggacagatctgggctgaagaattccagtgtgaggggcacgagtcccacctttcactctgcccagtagcaccccgccctgacgggacatgtagccacagcagggacgtcggcgtagtctgctcaagtgagacccagggaatgtgttcactttgttcccatgccatgaagagggtagggttaggtagtcacagacatctttttaaagccctgtctccttccaggatacacacaaatccgcttggtgaatggcaagaccccatgtgaaggaagagtggagctcaacattcttgggtcctgggggtccctctgcaactctcactgggacatggaagatgcccatgttttatgccagcagcttaaatgtggagttgccctttctatcccgggaggagcaccttttgggaaaggaagtgagcaggtctggaggcacatgtttcactgcactgggactgagaagcacatgggagattgttccgtcactgctctgggcgcatcactctgttcttcagggcaagtggcctctgtaatctgctcaggtaagagaataagggcagccagtgatgagccactcatgacggtgccttaagagtgggtgtacctaggagttcccattgtggctcagtggtaacaaactcgactggtatccatgagggtatgggtttgatccctggccttgctcaatgggttaaggatccagcattgctgtgagctgtggtataggttgcagactctgctcaggtcccatgttgctgtgattgtggtgtaggctgactgctgcagcttcaatttgacccctagcccgggaatttccataggccacacgtgcagcactaaggaaggaaaaaaagaaaaaaaaaaaaaaagagtgggtgtgcctatagtgaagaacagatgtaaaagggaagtgaaagggattcccccattctgagggattgtgagaagtgtgccagaatattaacttcatttgacttgttacagggaaagtaaacttgactttcacggacctcctagttacctggtgcttactatatgtcttctcagagtacctgattcattcccagcctggttgacccatccccctatctctatggctatgtttatccagagcacatctatctaacactccagctgatcttcctgacacagctgtggcaaccctggatcctttaaccaactgtgccaggctggagatcaaacctaagcctctgcagcaacccaagctgctgcagtcagatttttaaccccctgtgccactgtgggtatctccgatattttgtatcttctgtgactgagtggtttgctgtttgcagggaaccagagtcagacactatccccgtgcaattcatcatcctcggacccatcaagctctattatttcagaagaaaatggtgttgcctgcataggtgagaatcagtgaccaacctatgaaaatgatctcaatcctctgaaatgcattttattcatgttttatttcctctttgcagggagtggtcaacttcgcctggtcgatggaggtggtcgttgtgctgggagagtagaggtctatcatgagggctcctggggcaccatctgtgatgacagctgggacctgaatgatgcccatgtggtgtgcaaacagctgagctgtggatgggccattaatgccactggttctgctcattttggggaaggaacagggcccatttggctggatgagataaactgtaatggaaaagaatctcatatttggcaatgccactcacatggttgggggcggcacaattgcaggcataaggaggatgcaggagtcatctgctcgggtaagttctgcacatcacttcgggttacagtgatttaagaaacaactaaggtggggcaaagggtagtgaggcatatccatcagagcaaattccttgaaatacggactcagagggaaccattgtgagattgaggttcccagaggtgtggatttaatgaattagtgttacctcatgtacaaggtagtatactaccagaaagataaaaattcagaagcgagtttgcagcaaaactcatagggagaacttcttttataaataatatgaagctggatatttagtgcaccacctgatgaccactttattaataaataaagagttcctgttgtggcgcagcggaaatgaatccgacaaataatcatgagtttgcgggtttgatccctgacctcgctcagtgggttggggatctggtgttgccatgagctgtggtgtaggtcgcagatgctgcttggatcctgctttgctgtggctgtggtataggcttgtggctacagctccgatttgaccgctagcctgggaacctccatatgctgcgggggtggccctcaaaagaaaaataaataaataagtaaataaataagtagtttaaaaaggacaagaagaaatatatttggtgttatattctacagagacaaagataatcaccatgcccgattgatttttcaaggcatataaatgagacgtcatgggagcaaaaatggtcataatacaatgcccttgttttgtgtacatggtaagattttagaaagcattgtgaggtaaaaaagtgtactcagttataatatattggggaaaacagtactatgagaagtaaaaaaatctacatgccggaagttatttttttaatgtctcttttagagtcgcacatgcggcatatggaggttcccaggctaggggtcgaatcagagctatagccactggcttatggcacagccacaacaacactagatctgagccacatcagcgacctatactatagctcatggcaatgccagatccttaacctactgagccaagccatgggtcaaatccaggtcctcacggatcctaggcaaattcatttctgctgagccacgaagggaactcctcagaagtgattttgatgttactttcttttcatgacaaatctggtaaagtacatacacatagaaactgaagtgtcagaaagggaaatatttcattttaaggtaatgtatacaaaacagtggttttaccatctgagtatctcgctaaattttaactatcaaggacaattgccaaaaaaaaaaaaaaaagagagagagagagaacagaatagggttatgaagctaaaatcacagggttatgaagctaaaatcacagtaatttagggagaaaaaaatccaaagcatgtaattgataaaaggttctgagcctttgtttgagatttagaattcaacttagaaataccggtggtattttaaagcagtccataagtataaaatccaaggctaaaaaaccagaaggtatttgtagaacaaatatattttaataagctctaccaagtcatccagaagctattaaagaattactggtcactgacatagtgtacctgttttcaaggccattcttacatcagaataaagggagagcaccctctgaatcttcagaaaagatgtgaaagtgctaattctctatttcatcccagagttcatgtctctgagactgatcagtgaaaacagcagagagacctgtgcagggcgcctggaagttttttacaacggagcttggggcagcgttggcaagaatagcatgtctccagccacagtgggggtggtatgcaggcagctaggctgtgcagacagaggggacatcagccctgcatcttcagacaagacagtgtccaggcacatgtgggtggacaatgttcagtgtcctaaaggacctgacacactatggcagtgcccatcatctccatggaagaagagactggccagcccctcagaggagacatggatcacatgtgccagtgagtatccattctttagcgccactgttatcttctgatctacctaagcagaagttttataatctgtagttaatccctattctacctggatgatgggattcattctgtttaatttggtgtgcaggtattcagcatcagtgatcattttcccaaagaccatcatgctctgatggtcttctcaaaagttctaatcagttgcttcctccgtgaacagttgaggagcagagaatatgtaattcagaatttgactattgaatcatcccatttttctttcacatagtcttttgttgcactgaatataaggagagaagcagtcagaaagatcaatcctgaattatttctccattctacatctgttttaaatttcaaaaaaaaaaattgttataggtgatttacaatgtctgtcaatttctgctctacagcaaagtgacccagttatttacatatacattctgtttctcatatttttaaaccaggagatttctatctgcctggcggtttgagggaatttaacattatgcatttatgttaactttattcacctgatgttttctaagtcatactgagattcttatgcccaggatggaatacacctggtttgctggaaagacatgtgctttcataaagacgaattttggaaaaaatataaaatttaaaaggcccattaaataagcaaagttttaagagatttcaaaaaaaatttcatctctctcttttcctctttgacctcttgggcacgttcatcttctcaaatatgatcttggtgtttctgacttttcagacaaaataagacttcaagaaggaaacactaattgttctggacgtgtggagatctggtacggaggttcctggggcactgtgtgtgacgactcctgggaccttgaagatgctcaggtggtgtgccgacagctgggctgtggctcagctttggaggcaggaaaagaggccgcatttggccaggggactgggcccatatggctcaatgaagtgaagtgcaaggggaatgaaacctccttgtgggattgtcctgccagatcctggggccacagtgactgtggacacaaggaggatgctgctgtgacgtgttcaggtgagggcagagagtctggattgagcttggaagctctggcagcaaagagagggtgggcggtgacctgcattgggtaaagattggaaggtccagcctaaggatctggtggtggggggagacatgatgtttcagtctgaagaatgatgaaaacctgtgtggttacgcatgggccttcgccgaggaaagggacataactaccatgtatcctcctgcagagggaggaagaactaggggattctagttttgtgtgggaaggagcagtttacttggctcaggaggcactaaaggctcagataggaaacagagatctgttccattcttactcccagaactgattctcttctcttttctcctacagaaattgcaaagagccgagaatccctacatgccacaggtatatcaaaaagtttaagaacatgggacccattgtctgcattttgtggaatccctcttattaagacattctgggtcagaagttctgaggatttgacatttacttcagctatctgttatcttacccaagagagggatggtaactaggaacccaggtcttttagctaagacattatcacctcttgtgatgtttacttgttctcaggtcgctcatcttttgttgcacttgcaatctttggggtcattctgttggcctgtctcatcgcattcctcatttggactcagaagcgaagacagaggcagcggctctcaggtctgaacaaaattacggtctctctaatgtttctatgggagaagaagcctctctggataataaaacaaaaaaattacattcaagtatcagttggccagaaagagggaacctagaagaggtttaagcagtttctccgaaacagggaacaagaattcagagaagaaaaggcacattggctgtactgatgatacctgcactcgctatgtatgtttaatgggggacagtagagaattgatagtttagaaggagtatgcttatatggttctggatgaatcctgtatccccccaaacatttattttctcttactatatacttattactaatttaactcttctgtcaagccatgtgctaggttctgaagatggttcagacttggataaccaagtgcttttgttttcatggaatttccagtttagtggaagagataaatatgtaaacaaataaatggggggggggggggggggggggggggggggggggggggggggggggggggggggggggggggggggggggggggggggggggggggggggggggggggggggggggggggggggggggggggggggggggggggggggggggggggggggggggggggggggggggggggggggggggggggggggggggggggggggggggggggggggggggggggggggggggggggggggggggggggggggggggggggggggggggggggggggggggggggggggggggggggggggggggggggggggggggggggggggggggggggggggggggggggggggggggggggggggggggggggggggggggggggggggggggggggggggggggggggggggggggggggggggggggggggggggggggggggggggggggggggggggggggggggggggggggggggggggggggggggggggggggggggggggggggggggggggggggggggggggggggggggggggggggggggggggggggggggggggggggggggggggggggggggggggggggggggggggggggggggttggcgggcccccctcgaggtcgacggtatcgataagcttgatatcgaattcgtgagccagaggacgagactagagatggatgatgactacgttatgcttgcactgctggggaaaagcacacatagggagggaacgttttattatgacccagtccctaacctatgacctctgttatcagttttctcaggaggagagaattctgtccatcaaattcaataccgggagatgaattcttgcctgaaagcagatgaaacggatatgctaaatccctcaggtccgtgggttctttgaggggctgtagccctggggttcagatcagcagctgcagttgaggttgaggcatgctactttgcatagcagtagaaagaaatctcaactgtaataggaagcttgggatgcatatgaggaagaaaggcaagaatgaactacaaattattcttagggaagataaaaattgcagtcatggggagacctctggctgagagggccgtgattatttctgacagagggattatggagtagaatatgatggcttggaccttttttcactaaaacaagtcagtcttctcaaaggtagtttagcttttcatatatctttcacagtttcttccattcccatttcctgccattttcctttctctaacttttatttattatattttttcctaaaagtttaaattttctatatctttatcccttcagaagccatccctagtcacaggactagtctcatttcccattatgtaatgcttctttctctgtctgttgacttctatttagaaccagtgcactaaatctgcctttaggaacatacctctgctaggttgcaagaaatatcccattccccactcactctgtgaagactcaatgcttctcaatattccttacctcctgagagggacttgcctcacttctttaatccaagggactcgatttttgccaaaactaagtcaggaaaacctacataagacataggaaagacttgctgtgcttcttaaaccccactgtttgttttcctaattgtgaacagtatttttaaagttaacaagagagcttctaaggcacttgaggggagatctgatttatttcccagtaattattttcttcctttcagaaaattccactgaataagatggttttaacggatgtgggactaatttttgtgtctaaatctcttcctatttctggatgaaaaaaaggagaccactctgaagtacaatgaaaaggaaaatgggaattataacctggtgaggtgagtaggaagaatttattcatcattgctgaaaacaggtacattccttttgaaagttgagaactcctctggtattagaaaaaaaaaaagaacgtatatacacatatatttccatgtctatgtttatgtttgtaaatccatattcagaatatgcaacaactttttataactatgacttcagtccatcttttagttacatatatattctaaacaacaactattgctaagagaagctgggtaagtaaatgtgaataaatcttctaaagatattacaggaagttcctgctgcggctcagtgggttaaagacttgatgtctttgtgaagatgagggctcgagccctggcctcactcagtgagttaaggatctagcattgctgtaagctgcagcgtaggttgcagatagggctcagatccagtgttgctgtggctgtggcctcagttgcagctctgattcaacccttaggcgaggaacttccatatgcagcaaatgtggccattaaaaaaaaaaaaaacattataggagtcatttcataaaagagataagacgtttctatagttatatagtgcatactctggtaaagatagtataggatactataggaatatagaaagcttgcctatgaaaatttgggaagattgtggaaaagacatctcaaaatatggcatagaaaagaatcatatctttgaggaacagtaagtttttcattcaaaaccgtgtattgaacatacttgtggtgacaagtggtgtcctgagtactaaaaattcagtgataaaagatgctcttgacaaagacatggctgttgaatagaaggtctcactgtcaatgtgtgggaattatggacagcctatgtggacacagggaatagatgagactctaggctggaaggctgcattgagcccaataatgaatggtcctgtctgatatatttcatgctcatattttattttagggactattggggaggtggtgggttttggaagattaagctgaggcaagacacaatcagattgccttttataatttactttcaggaggaaagtctaactaaaaaaagaattcgatatcaagcttatcgataccgtcgacctcgaggaggcccgcctgcccttttggggggggggggggggggggggggggggggggggggggggggggggggggggggggggggggggggggggggggggggggggggggggggggggggggggcagcaccaattttattattggcgggaataaagagaaaaatgtaatttcaaagattgctgttggaaatgaggggtgtggtagcttttggagaaagcattctggagacttctattaattttttttttttaagtgcttcaaagatcctttgatccaacaattctactcctaaaaatttcttccatacagataaagccatttgtctgtatataacaaatagaagagaattcctttttgcagccttgttagtagtgcccccaaactggaaacaaagtgaatatcagtcagtggggtagcggctggaaaaattttagtgcacccaaccaacaaagaaaaaccatgcacaaaaattcaataaatatcatctcacttttgtgttcatgttattgaatataattaaacataatgtttacatctataaaattatcatatgtatacatgtaaagaaacattaaaacatttttaacagactgtaaacttgaggactgtgaatgacttttgattgataatctcaaacatatggatactattctgatgtaataaataatgattaaattttttccctaaagagtaatcactactgaatcgttgcctcagaatcatatggaggtgcttttaaaaaaggcatttctgcactgttgttctctggaatagaagtaattcttatgtacactgaagtttgaaaatcattgcatttaagtgttctgttcaggaaagtagtgtgctttttaatatttgtgagtgaatgagtaacacaatacattatatcacattttaatgtaattctacacatgtgcatatgaagagaaaagtaacatttttttctatttatgtctttagttcagcctttaagataccttgatgaagacctggactattgaatgagcaagaatctgcctcttacactgaagattacaatacagtcctctgtctcctggtattccaaagactgctgttgaatttctaaaaaatagattggtgaatgtgactactcaaagttgtatgtaagactttcaagggcattaaataaaaaagaatattgctgattcttgttcttgattttctgaatttctgaatctcttattgggcttctaatttaaaaaaaaatatctgggcgcccgcagatatcgaactcttgggcagtgtgaccaaacgaagacatatccaatcaagcatgcaaatggaccagcccactgtactagcacgctgtggcagccaatctgaccgagaaagcagacaaccgcagggagcaacg

SEQ ID NO: 16 - DNA, 55 bp, Sus scrofa
  source 1..55: mol_type = other DNA
ggtcgccaccatggtgagcaagggcgaggagctgttcaccggggtggtgcccatc

SEQ ID NO: 17 - DNA, 54 bp, Sus scrofa
  source 1..54: mol_type = other DNA
ggtcgccaccatggccatgagcaagggcgaggagctgttcaccggggtggtgcc

SEQ ID NO: 18 - DNA, 48 bp, Sus scrofa
  source 1..48: mol_type = other DNA
ggtcgccaccatggtgagcaagggcgaggagctgttcaccggggtggt

SEQ ID NO: 19 - DNA, 55 bp, Sus scrofa
  source 1..55: mol_type = other DNA
ggtcgccaccatggttgagcaagggcgaggagctgttcaccggggtggtgcccat

SEQ ID NO: 20 - DNA, 43 bp, Sus scrofa
  source 1..43: mol_type = other DNA
tgcagggaactacagtgcggcactgtggtttccctcctggggg

SEQ ID NO: 21 - DNA, 60 bp, Sus scrofa
  source 1..60: mol_type = other DNA
tgcagggaactacagtgcggcactgtaaaccactactactgtggtttccctcctgggggg

SEQ ID NO: 22 - DNA, 41 bp, Sus scrofa
  source 1..41: mol_type = other DNA
tgcagggaactacagtgcggctgtggtttccctcctggggg

SEQ ID NO: 23 - DNA, 46 bp, Sus scrofa
  source 1..46: mol_type = other DNA
tgcagggaactacagtgcggaactactgtggtttccctcctggggg

SEQ ID NO: 24 - DNA, 31 bp, Sus scrofa
  source 1..31: mol_type = other DNA
gaaacccaggctggttggaggggacattccc

SEQ ID NO: 25 - DNA, 24 bp, Sus scrofa
  source 1..24: mol_type = other DNA
gaaacccaggctggggacattccc

SEQ ID NO: 26 - DNA, 13 bp, Sus scrofa
  source 1..13: mol_type = other DNA
aggggacattccc

SEQ ID NO: 27 - DNA, 13 bp, Sus scrofa
  source 1..13: mol_type = other DNA
gaaacccattccc

SEQ ID NO: 28 - DNA, 31 bp, Sus scrofa
  source 1..31: mol_type = other DNA
ggtcgccaccatggtgagcaagggcgaggag

SEQ ID NO: 29 - DNA, 32 bp, Sus scrofa
  source 1..32: mol_type = other DNA
ggtcgccaccatggctgagcaagggcgaggag

SEQ ID NO: 30 - DNA, 29 bp, Sus scrofa
  source 1..29: mol_type = other DNA
ggtcgccaccatggtgagagggcgaggag

SEQ ID NO: 31 - DNA, 32 bp, Sus scrofa
  source 1..32: mol_type = other DNA
ggtcgccaccatggttgagcaagggcgaggag

SEQ ID NO: 32 - DNA, 48 bp, Sus scrofa
  source 1..48: mol_type = other DNA
ggtcgccaccatggtgagcaagggcgaggagaacccaggctggttgga

SEQ ID NO: 33 - DNA, 49 bp, Sus scrofa
  source 1..49: mol_type = other DNA
tgctgtgcagggaactacagtgcggcactgtggtttccctcctgggggg

SEQ ID NO: 34 - DNA, 38 bp, Sus scrofa
  source 1..38: mol_type = other DNA
tgctgtgcagggaactctgtggtttccctcctgggggg

SEQ ID NO: 35 - DNA, 22 bp, Sus scrofa
  source 1..22: mol_type = other DNA
ctgtggtttccctcctgggggg

SEQ ID NO: 36 - DNA, 23 bp, Sus scrofa
  source 1..23: mol_type = other DNA
actgtggtttccctcctgggggg

SEQ ID NO: 37 - DNA, 50 bp, Sus scrofa
  source 1..50: mol_type = other DNA
tgctgtgcagggaactacagtgcggcaactgtggtttccctcctgggggg

SEQ ID NO: 38 - DNA, 10 bp, Sus scrofa
  source 1..10: mol_type = other DNA
tcctgggggg

SEQ ID NO: 39 - skipped

SEQ ID NO: 40 - DNA, 52 bp, Sus scrofa
  source 1..52: mol_type = other DNA
agagagcagagccagcgactcgcccagcgacatggggtacctgccgtttgtg

SEQ ID NO: 41 - DNA, 33 bp, Sus scrofa
  source 1..33: mol_type = other DNA
agagagcagagccagcgactcgcccagcgagat

SEQ ID NO: 42 - DNA, 30 bp, Sus scrofa
  source 1..30: mol_type = other DNA
agagagcagagccagcgactcgcccagcga

SEQ ID NO: 43 - DNA, 50 bp, Sus scrofa
  source 1..50: mol_type = other DNA
agagccagcctcgcccagcaggggtaccatggggtacctgccgtttgtgt

SEQ ID NO: 44 - DNA, 53 bp, Sus scrofa
  source 1..53: mol_type = other DNA
agagagcagagccagcgactcgcccagcgagcagtgggtacctgccgtttgtg

SEQ ID NO: 45 - DNA, 53 bp, Sus scrofa
  source 1..53: mol_type = other DNA
agagagcagagccagcgactcgcccagcgatcagtgggtacctgccgtttgtg

SEQ ID NO: 46 - DNA, 53 bp, Sus scrofa
  source 1..53: mol_type = other DNA
agagagcagagccagcgactcgcccagcgaacatggggtacctgccgtttgtg

SEQ ID NO: 47 - DNA, 4990 bp, Sus scrofa
  source 1..4990: mol_type = other DNA
tatagatgacaaggctttgtgtctgataggggccagcgaactcagtaaagagggaagatgagaaagataatggcaagaatttatccctgaagtgtagttttgacaaaccagtcacaaagaggtctaagaaattttggtcacaaagttgttttgaatcccaggcattttatttgcaatgattgcatatgttctggaaaggacatctgaacctaagaaatagttcatttgcattgtgttatattttactaaggtctgagaaataatcttgagatgagaatgaactctacttcttcagagtctggaaggaataaattatgaaaatgtattaatgcttctttaaaccatattgtatatttatctattactaaacaaaaagaagtagctctatttatttatttatttatttatttatttatgtcttttgtctctttagggccacacctgtggcatatggaggttcccaggctagaggtccaattggagatgtagcagccagcctatgccagagccaccgcaacacgggatctgagccacgtctgtgacttacaccacagctcacagcaacgcctgatcctcaacccactgagcgaggccagggatcgaacccatgtcctcatggatgctagttgggttcgttaactgctgagccatgatgggaactccaaattaattatttcttatatttgttcttcatatattcatttctatagaaagaaataaatacagattcagttaatgatggcaggtaaaagcttaacttattaatcaaaggagttaatccaggcacaaaaattcaattcatggctctctgttaaaatttaggtataggtttagcaggaagaaaaggttagtagatgcagactattacatttagaatggatggacaatgaagtcctactatacagcacagggaactatatccaatctcttgggatagaatatgatggaagacaaaatcagaacaagagagtatatatatatgtgtgtgtgtgtgtgtgtgtgtgtgtgtgtgtgtgtgtgtgtgtgactgggtcaccctgcggcacagcagaaattggcagaacattgtaaatcaactatactttaataggaaaaatacttttaagggctaaatttccaatattctaaccatgtacacagagtaaatgtcataaggatgccagtctgtgtagagattgatgtgttactagcagattcatgaaataaaggctgaggatgtagtccccaagtcacttctgagtggaagaatttctcctttgtcctggactcaaatattttaggataaaggaaaaaagaagatatttatagaagggacttgttttcaagtacttgacaaaatttcaccattaaagagaaatttgtgggagttcccatcgtggctcagtggaaacaaatccaactaggaaccatgaggttgtgggtttgatccctggcctcactcagtgggttaaggatccggtgttgccgtgagctgtggtgtaggttgcagacacggttctgatcctgcgttgctgtggctgtggctgtggtgtaggccagcagcaaacagctctgattagacccctagcctggaaacctccatatgccacaggtgcagccctaaaaagacaaaaaaagagaaaagacaaaaaaaaaaaaaaaaaaaaaaaaaaaaaaaaaaaaaaaaaaaagaacccccagaggtatttatttgtttttgccttttttcactgactgttctttgtttgtttgtttgagactgatctagaagactagagattacaagaaatatggatttggctcactctaagaaactgctttcattccaaggtttgggtctatccaaaagtggaatagaatcatatgaatactagtttatgagtatttagtgagaggaatttcaagctcaaataatgattcagcaagattaaattaaggagggaattttccttgtggctgagtgggttaaggacccaatgttgtctctgtgaggatgtaggttccatcctgggctttgctcattaggttaaggatctggcattgctgcagctcagacccagtgctgccctggttgtggcttaggccaaagctgcagctccaattcaatctctggcctgggaacctccatgtgctacaaggtgcggccttaaaaggaaaaaaaaaaaattaaatcaaggactcaagagtctttcattatttgtgttgtggaagctatatttgttttaaagtcttagttgtgtttagaaagcaagatgttcttcaactcaaatttgggagggaacttgtttcatacatttttaatggataagtggcaaaattttcatgctgaggtgatctatagtgttgtaatgcagaatatagtcagatcttgaacattttaggaagttggtgagggccaattgtgtatctgtgccatgctgataagaatgtcaagggatcacaagaattcgtgttatttgacagcagtcatctttaaaaggcatttgagaaagtccaatttcaaatgcatttcctttctttaaaagataaattgaagaaaataagtctttatttcccaagtaaattgaattgcctctcagtctgttaaaagaaactcttaccttgatgattgcgctcttaacctggcaaagattgtctttaaaatctgagctccatgtcttctgctttatttctggtgtgcctttgactccagattacagtaaatggaggactgagtatagggctaaaaagtagagagaatggatgcatattatctgtggtctccaatgtgatgaatgaagtaggcaaatactcaaaggaaagagaaagcatgctccaagaattatgggttccagaaggcaaagtcccagaattgtctccagggaaggacagggaggtctagaatcggctaagcccactgtaggcagaaaaaccaagaggcatgaatggcttccctttctcacttttcactctctggcttactcctatcatgaaggaaaatattggaatcatattctccctcaccgaaatgctatttttcagcccacaggaaacccaggctggttggaggggacattccctgctctggtcgtgttgaagtacaacatggagacacgtggggcaccgtctgtgattctgacttctctctggaggcggccagcgtgctgtgcagggaactacagtgcggcactgtggtttccctcctggggggagctcactttggagaaggaagtggacagatctgggctgaagaattccagtgtgaggggcacgagtcccacctttcactctgcccagtagcaccccgccctgacgggacatgtagccacagcagggacgtcggcgtagtctgctcaagtgagacccagggaatgtgttcactttgttcccatgccatgaagagggtagggttaggtagtcacagacatctttttaaagccctgtctccttccaggatacacacaaatccgcttggtgaatggcaagaccccatgtgaaggaagagtggagctcaacattcttgggtcctgggggtccctctgcaactctcactgggacatggaagatgcccatgttttatgccagcagcttaaatgtggagttgccctttctatcccgggaggagcaccttttgggaaaggaagtgagcaggtctggaggcacatgtttcactgcactgggactgagaagcacatgggagattgttccgtcactgctctgggcgcatcactctgttcttcagggcaagtggcctctgtaatctgctcaggtaagagaataagggcagccagtgatgagccactcatgacggtgccttaagagtgggtgtacctaggagttcccattgtggctcagtggtaacaaactcgactggtatccatgagggtatgggtttgatccctggccttgctcaatgggttaaggatccagcattgctgtgagctgtggtataggttgcagactctgctcaggtcccatgttgctgtgattgtggtgtaggctgactgctgcagcttcaatttgacccctagcccgggaatttccataggccacacgtgcagcactaaggaaggaaaaaaagaaaaaaaaaaaaaaagagtgggtgtgcctatagtgaagaacagatgtaaaagggaagtgaaagggattcccccattctgagggattgtgagaagtgtgccagaatattaacttcatttgacttgttacagggaaagtaaacttgactttcacggacctcctagttacctggtgcttactatatgtcttctcagagtacctgattcattcccagcctggttgacccatccccctatctctatggctatgtttatccagagcacatctatctaacactccagctgatcttcctgacacagctgtggcaaccctggatcctttaaccaactgtgccaggctggagatcaaacctaagcctctgcagcaacccaagctgctgcagtcagatttttaaccccctgtgccactgtgggtatctccgatattttgtatcttctgtgactgagtggtttgctgtttgcagggaaccagagtcagacactatccccgtgcaattcatcatcctcggacccatcaagctctattatttcagaagaaaatggtgttgcctgcataggtgagaatcagtgaccaacctatgaaaatgatctcaatcctctgaaatgcattttattcatgttttatttcctctttgcagggagtggtcaacttcgcctggtcgatggaggtggtcgttgtgctgggagagtagaggtctatcatgagggctcctggggcaccatctgtgatgacagctgggacctgaatgatgcccatgtggtgtgcaaacagctgagctgtggatgggccattaatgccactggttctgctcattttggggaaggaacagggcccatttggctggatgagataaactgtaatggaaaagaatctcatatttggcaatgccactcacatggttgggggcggcacaattgcaggcataaggaggatgcaggagtcatctgctcgg

SEQ ID NO: 48 - DNA, 24 bp, synthetic construct
  misc_feature 1..24: note = Synthetic oligonucleotide
  source 1..24: mol_type = other DNA
caccggaaacccaggctggttgga

SEQ ID NO: 49 - DNA, 24 bp, synthetic construct
  misc_feature 1..24: note = Synthetic oligonucleotide
  source 1..24: mol_type = other DNA
aaactccaaccagcctgggtttcc

SEQ ID NO: 50 - DNA, 24 bp, synthetic construct
  misc_feature 1..24: note = Synthetic oligonucleotide
  source 1..24: mol_type = other DNA
caccggaactacagtgcggcactg

SEQ ID NO: 51 - DNA, 24 bp, synthetic construct
  misc_feature 1..24: note = Synthetic oligonucleotide
  source 1..24: mol_type = other DNA
aaaccagtgccgcactgtagttcc

SEQ ID NO: 52 - DNA, 25 bp, synthetic construct
  misc_feature 1..25: note = Synthetic oligonucleotide
  source 1..25: mol_type = other DNA
caccgcagtagcaccccgccctgac

SEQ ID NO: 53 - DNA, 25 bp, synthetic construct
  misc_feature 1..25: note = Synthetic oligonucleotide
  source 1..25: mol_type = other DNA
aaacgtcagggcggggtgctactgc

SEQ ID NO: 54 - DNA, 25 bp, synthetic construct
  misc_feature 1..25: note = Synthetic oligonucleotide
  source 1..25: mol_type = other DNA
caccgtgtagccacagcagggacgt

SEQ ID NO: 55 - DNA, 25 bp, synthetic construct
  misc_feature 1..25: note = Synthetic oligonucleotide
  source 1..25: mol_type = other DNA
aaacacgtccctgctgtggctacac

SEQ ID NO: 56 - DNA, 25 bp, synthetic construct
  misc_feature 1..25: note = Synthetic oligonucleotide
  source 1..25: mol_type = other DNA
caccgccagcctcgcccagcgacat

SEQ ID NO: 57 - DNA, 25 bp, synthetic construct
  misc_feature 1..25: note = Synthetic oligonucleotide
  source 1..25: mol_type = other DNA
aaacatgtcgctgggcgaggctggc

SEQ ID NO: 58 - DNA, 25 bp, synthetic construct
  misc_feature 1..25: note = Synthetic oligonucleotide
  source 1..25: mol_type = other DNA
caccgcagctgcagcatatatttaa

SEQ ID NO: 59 - DNA, 25 bp, synthetic construct
  misc_feature 1..25: note = Synthetic oligonucleotide
  source 1..25: mol_type = other DNA
aaacttaaatatatgctgcagctgc

SEQ ID NO: 60 - DNA, 25 bp, synthetic construct
  misc_feature 1..25: note = Synthetic oligonucleotide
  source 1..25: mol_type = other DNA
caccgctttcatttatctgaactca

SEQ ID NO: 61 - DNA, 25 bp, synthetic construct
  misc_feature 1..25: note = Synthetic oligonucleotide
  source 1..25: mol_type = other DNA
aaactgagttcagataaatgaaagc

SEQ ID NO: 62 - DNA, 25 bp, synthetic construct
  misc_feature 1..25: note = Synthetic oligonucleotide
  source 1..25: mol_type = other DNA
caccgttatctgaactcagggtccc

SEQ ID NO: 63 - DNA, 25 bp, synthetic construct
  misc_feature 1..25: note = Synthetic oligonucleotide
  source 1..25: mol_type = other DNA
aaacgggaccctgagttcagataac

SEQ ID NO: 64 - DNA, 25 bp, synthetic construct
  misc_feature 1..25: note = Synthetic oligonucleotide
  source 1..25: mol_type = other DNA
caccgctcctcgcccttgctcacca

SEQ ID NO: 65 - DNA, 25 bp, synthetic construct
  misc_feature 1..25: note = Synthetic oligonucleotide
  source 1..25: mol_type = other DNA
aaactggtgagcaagggcgaggagc

SEQ ID NO: 66 - DNA, 25 bp, synthetic construct
  misc_feature 1..25: note = Synthetic oligonucleotide
  source 1..25: mol_type = other DNA
caccggaccaggatgggcaccaccc

SEQ ID NO: 67 - DNA, 25 bp, synthetic construct
  misc_feature 1..25: note = Synthetic oligonucleotide
  source 1..25: mol_type = other DNA
aaacgggtggtgcccatcctggtcc

SEQ ID NO: 68 - DNA, 24 bp, synthetic construct
  misc_feature 1..24: note = Synthetic oligonucleotide
  source 1..24: mol_type = other DNA
ttgttggaaggctcactgtccttg

SEQ ID NO: 69 - DNA, 20 bp, synthetic construct
  misc_feature 1..20: note = Synthetic oligonucleotide
  source 1..20: mol_type = other DNA
acaactaaggtggggcaaag

SEQ ID NO: 70 - DNA, 24 bp, synthetic construct
  misc_feature 1..24: note = Synthetic oligonucleotide
  source 1..24: mol_type = other DNA
ttgttggaaggctcactgtccttg

SEQ ID NO: 71 - DNA, 23 bp, synthetic construct
  misc_feature 1..23: note = Synthetic oligonucleotide
  source 1..23: mol_type = other DNA
ggagctcaacattcttgggtcct

SEQ ID NO: 72 - DNA, 23 bp, synthetic construct
  misc_feature 1..23: note = Synthetic oligonucleotide
  source 1..23: mol_type = other DNA
ggcaaaattttcatgctgaggtg

SEQ ID NO: 73 - DNA, 23 bp, synthetic construct
  misc_feature 1..23: note = Synthetic oligonucleotide
  source 1..23: mol_type = other DNA
gcacatcacttcgggttacagtg

SEQ ID NO: 74 - DNA, 23 bp, synthetic construct
  misc_feature 1..23: note = Synthetic oligonucleotide
  source 1..23: mol_type = other DNA
cccaagtatcttcagttctgcag

SEQ ID NO: 75 - DNA, 23 bp, synthetic construct
  misc_feature 1..23: note = Synthetic oligonucleotide
  source 1..23: mol_type = other DNA
tacaggtaggagagcctgttttg

SEQ ID NO: 76 - DNA, 23 bp, synthetic construct
  misc_feature 1..23: note = Synthetic oligonucleotide
  source 1..23: mol_type = other DNA
cccaagtatcttcagttctgcag

SEQ ID NO: 77 - DNA, 23 bp, synthetic construct
  misc_feature 1..23: note = Synthetic oligonucleotide
  source 1..23: mol_type = other DNA
ctcaaaaggatgtaaaccctgga

SEQ ID NO: 78 - DNA, 22 bp, synthetic construct
  misc_feature 1..22: note = Synthetic oligonucleotide
  source 1..22: mol_type = other DNA
tgttgatgtggtttgtttgccc

SEQ ID NO: 79 - DNA, 23 bp, synthetic construct
  misc_feature 1..23: note = Synthetic oligonucleotide
  source 1..23: mol_type = other DNA
tacaggtaggagagcctgttttg

SEQ ID NO: 80 - DNA, 23 bp, synthetic construct
  misc_feature 1..23: note = Synthetic oligonucleotide
  source 1..23: mol_type = other DNA
ggaggtctagaatcggctaagcc

SEQ ID NO: 81 - DNA, 20 bp, synthetic construct
  misc_feature 1..20: note = Synthetic oligonucleotide
  source 1..20: mol_type = other DNA
ggctacatgtcccgtcaggg

SEQ ID NO: 82 - DNA, 21 bp, synthetic construct
  misc_feature 1..21: note = Synthetic oligonucleotide
  source 1..21: mol_type = other DNA
gcaggccactaggcagatgaa

SEQ ID NO: 83 - DNA, 23 bp, synthetic construct
  misc_feature 1..23: note = Synthetic oligonucleotide
  source 1..23: mol_type = other DNA
gagctgacacccaagaagttcct

SEQ ID NO: 84 - DNA, 22 bp, synthetic construct
  misc_feature 1..22: note = Synthetic oligonucleotide
  source 1..22: mol_type = other DNA
ggctctagagcctctgctaacc

SEQ ID NO: 85 - DNA, 22 bp, synthetic construct
  misc_feature 1..22: note = Synthetic oligonucleotide
  source 1..22: mol_type = other DNA
ggacttgaagaagtcgtgctgc

SEQ ID NO: 86 - DNA, 44 bp, synthetic construct
  misc_feature 1..44: note = Synthetic oligonucleotide
  source 1..44: mol_type = other DNA
taatacgactcactatagggagaatggactataaggaccacgac

SEQ ID NO: 87 - DNA, 21 bp, synthetic construct
  misc_feature 1..21: note = Synthetic oligonucleotide
  source 1..21: mol_type = other DNA
gcgagctctaggaattcttac

SEQ ID NO: 88 - DNA, 40 bp, synthetic construct
  misc_feature 1..40: note = Synthetic oligonucleotide
  source 1..40: mol_type = other DNA
ttaatacgactcactataggctcctcgcccttgctcacca

SEQ ID NO: 89 - DNA, 20 bp, synthetic construct
  misc_feature 1..20: note = Synthetic oligonucleotide
  source 1..20: mol_type = other DNA
aaaagcaccgactcggtgcc

SEQ ID NO: 90 - DNA, 38 bp, synthetic construct
  misc_feature 1..38: note = Synthetic oligonucleotide
  source 1..38: mol_type = other DNA
ttaatacgactcactataggaaacccaggctggttgga

SEQ ID NO: 91 - DNA, 20 bp, synthetic construct
  misc_feature 1..20: note = Synthetic oligonucleotide
  source 1..20: mol_type = other DNA
aaaagcaccgactcggtgcc

SEQ ID NO: 92 - DNA, 38 bp, synthetic construct
  misc_feature 1..38: note = Synthetic oligonucleotide
  source 1..38: mol_type = other DNA
ttaatacgactcactataggaactacagtgcggcactg

SEQ ID NO: 93 - DNA, 20 bp, synthetic construct
  misc_feature 1..20: note = Synthetic oligonucleotide
  source 1..20: mol_type = other DNA
aaaagcaccgactcggtgcc

SEQ ID NO: 94 - DNA, 40 bp, synthetic construct
  misc_feature 1..40: note = Synthetic oligonucleotide
  source 1..40: mol_type = other DNA
ttaatacgactcactataggccagcctcgcccagcgacat

SEQ ID NO: 95 - DNA, 20 bp, synthetic construct
  misc_feature 1..20: note = Synthetic oligonucleotide
  source 1..20: mol_type = other DNA
aaaagcaccgactcggtgcc

SEQ ID NO: 96 - DNA, 40 bp, synthetic construct
  misc_feature 1..40: note = Synthetic oligonucleotide
  source 1..40: mol_type = other DNA
ttaatacgactcactataggcagctgcagcatatatttaa

SEQ ID NO: 97 - DNA, 20 bp, synthetic construct
  misc_feature 1..20: note = Synthetic oligonucleotide
  source 1..20: mol_type = other DNA
aaaagcaccgactcggtgcc

SEQ ID NO: 98 - DNA, 3484 bp, Sus scrofa
  source 1..3484: mol_type = other DNA
tatagatgacaaggctttgtgtctgataggggccagcgaactcagtaaagagggaagatgagaaagataatggcaagaatttatccctgaagtgtagttttgacaaaccagtcacaaagaggtctaagaaattttggtcacaaagttgttttgaatcccaggcattttatttgcaatgattgcatatgttctggaaaggacatctgaacctaagaaatagttcatttgcattgtgttatattttactaaggtctgagaaataatcttgagatgagaatgaactctacttcttcagagtctggaaggaataaattatgaaaatgtattaatgcttctttaaaccatattgtatatttatctattactaaacaaaaagaagtagctctatttatttatttatttatttatttatttatgtcttttgtctctttagggccacacctgtggcatatggaggttcccaggctagaggtccaattggagatgtagcagccagcctatgccagagccaccgcaacacgggatctgagccacgtctgtgacttacaccacagctcacagcaacgcctgatcctcaacccactgagcgaggccagggatcgaacccatgtcctcatggatgctagttgggttcgttaactgctgagccatgatgggaactccaaattaattatttcttatatttgttcttcatatattcatttctatagaaagaaataaatacagattcagttaatgatggcaggtaaaagcttaacttattaatcaaaggagttaatccaggcacaaaaattcaattcatggctctctgttaaaatttaggtataggtttagcaggaagaaaaggttagtagatgcagactattacatttagaatggatggacaatgaagtcctactatacagcacagggaactatatccaatctcttgggatagaatatgatggaagacaaaatcagaacaagagagtatatatatatgtgtgtgtgtgtgtgtgtgtgtgtgtgtgtgtgtgtgtgtgtgtgactgggtcaccctgcggcacagcagaaattggcagaacattgtaaatcaactatactttaataggaaaaatacttttaagggctaaatttccaatattctaaccatgtacacagagtaaatgtcataaggatgccagtctgtgtagagattgatgtgttactagcagattcatgaaataaaggctgaggatgtagtccccaagtcacttctgagtggaagaatttctcctttgtcctggactcaaatattttaggataaaggaaaaaagaagatatttatagaagggacttgttttcaagtacttgacaaaatttcaccattaaagagaaatttgtgggagttcccatcgtggctcagtggaaacaaatccaactaggaaccatgaggttgtgggtttgatccctggcctcactcagtgggttaaggatccggtgttgccgtgagctgtggtgtaggttgcagacacggttctgatcctgcgttgctgtggctgtggcacattccctgctctggtcgtgttgaagtacaacatggagacacgtggggcaccgtctgtgattctgacttctctctggaggcggccagcgtgctgtgcagggaactacagtgcggcactgtggtttccctcctggggggagctcactttggagaaggaagtggacagatctgggctgaagaattccagtgtgaggggcacgagtcccacctttcactctgcccagtagcaccccgccctgacgggacatgtagccacagcagggacgtcggcgtagtctgctcaagtgagacccagggaatgtgttcactttgttcccatgccatgaagagggtagggttaggtagtcacagacatctttttaaagccctgtctccttccaggatacacacaaatccgcttggtgaatggcaagaccccatgtgaaggaagagtggagctcaacattcttgggtcctgggggtccctctgcaactctcactgggacatggaagatgcccatgttttatgccagcagcttaaatgtggagttgccctttctatcccgggaggagcaccttttgggaaaggaagtgagcaggtctggaggcacatgtttcactgcactgggactgagaagcacatgggagattgttccgtcactgctctgggcgcatcactctgttcttcagggcaagtggcctctgtaatctgctcaggtaagagaataagggcagccagtgatgagccactcatgacggtgccttaagagtgggtgtacctaggagttcccattgtggctcagtggtaacaaactcgactggtatccatgagggtatgggtttgatccctggccttgctcaatgggttaaggatccagcattgctgtgagctgtggtataggttgcagactctgctcaggtcccatgttgctgtgattgtggtgtaggctgactgctgcagcttcaatttgacccctagcccgggaatttccataggccacacgtgcagcactaaggaaggaaaaaaagaaaaaaaaaaaaaaagagtgggtgtgcctatagtgaagaacagatgtaaaagggaagtgaaagggattcccccattctgagggattgtgagaagtgtgccagaatattaacttcatttgacttgttacagggaaagtaaacttgactttcacggacctcctagttacctggtgcttactatatgtcttctcagagtacctgattcattcccagcctggttgacccatccccctatctctatggctatgtttatccagagcacatctatctaacactccagctgatcttcctgacacagctgtggcaaccctggatcctttaaccaactgtgccaggctggagatcaaacctaagcctctgcagcaacccaagctgctgcagtcagatttttaaccccctgtgccactgtgggtatctccgatattttgtatcttctgtgactgagtggtttgctgtttgcagggaaccagagtcagacactatccccgtgcaattcatcatcctcggacccatcaagctctattatttcagaagaaaatggtgttgcctgcataggtgagaatcagtgaccaacctatgaaaatgatctcaatcctctgaaatgcattttattcatgttttatttcctctttgcagggagtggtcaacttcgcctggtcgatggaggtggtcgttgtgctgggagagtagaggtctatcatgagggctcctggggcaccatctgtgatgacagctgggacctgaatgatgcccatgtggtgtgcaaacagctgagctgtggatgggccattaatgccactggttctgctcattttggggaaggaacagggcccatttggctggatgagataaactgtaatggaaaagaatctcatatttggcaatgccactcacatggttgggggcggcacaattgcaggcataaggaggatgcaggagtcatctgctcgg

SEQ ID NO: 99 - DNA, 4997 bp, Sus scrofa
  source 1..4997: mol_type = other DNA
tatagatgacaaggctttgtgtctgataggggccagcgaactcagtaaagagggaagatgagaaagataatggcaagaatttatccctgaagtgtagttttgacaaaccagtcacaaagaggtctaagaaattttggtcacaaagttgttttgaatcccaggcattttatttgcaatgattgcatatgttctggaaaggacatctgaacctaagaaatagttcatttgcattgtgttatattttactaaggtctgagaaataatcttgagatgagaatgaactctacttcttcagagtctggaaggaataaattatgaaaatgtattaatgcttctttaaaccatattgtatatttatctattactaaacaaaaagaagtagctctatttatttatttatttatttatttatttatgtcttttgtctctttagggccacacctgtggcatatggaggttcccaggctagaggtccaattggagatgtagcagccagcctatgccagagccaccgcaacacgggatctgagccacgtctgtgacttacaccacagctcacagcaacgcctgatcctcaacccactgagcgaggccagggatcgaacccatgtcctcatggatgctagttgggttcgttaactgctgagccatgatgggaactccaaattaattatttcttatatttgttcttcatatattcatttctatagaaagaaataaatacagattcagttaatgatggcaggtaaaagcttaacttattaatcaaaggagttaatccaggcacaaaaattcaattcatggctctctgttaaaatttaggtataggtttagcaggaagaaaaggttagtagatgcagactattacatttagaatggatggacaatgaagtcctactatacagcacagggaactatatccaatctcttgggatagaatatgatggaagacaaaatcagaacaagagagtatatatatatgtgtgtgtgtgtgtgtgtgtgtgtgtgtgtgtgtgtgtgtgtgtgactgggtcaccctgcggcacagcagaaattggcagaacattgtaaatcaactatactttaataggaaaaatacttttaagggctaaatttccaatattctaaccatgtacacagagtaaatgtcataaggatgccagtctgtgtagagattgatgtgttactagcagattcatgaaataaaggctgaggatgtagtccccaagtcacttctgagtggaagaatttctcctttgtcctggactcaaatattttaggataaaggaaaaaagaagatatttatagaagggacttgttttcaagtacttgacaaaatttcaccattaaagagaaatttgtgggagttcccatcgtggctcagtggaaacaaatccaactaggaaccatgaggttgtgggtttgatccctggcctcactcagtgggttaaggatccggtgttgccgtgagctgtggtgtaggttgcagacacggttctgatcctgcgttgctgtggctgtggctgtggtgtaggccagcagcaaacagctctgattagacccctagcctggaaacctccatatgccacaggtgcagccctaaaaagacaaaaaaagagaaaagacaaaaaaaaaaaaaaaaaaaaaaaaaaaaaaaaaaaaaaaaaaaagaacccccagaggtatttatttgtttttgccttttttcactgactgttctttgtttgtttgtttgagactgatctagaagactagagattacaagaaatatggatttggctcactctaagaaactgctttcattccaaggtttgggtctatccaaaagtggaatagaatcatatgaatactagtttatgagtatttagtgagaggaatttcaagctcaaataatgattcagcaagattaaattaaggagggaattttccttgtggctgagtgggttaaggacccaatgttgtctctgtgaggatgtaggttccatcctgggctttgctcattaggttaaggatctggcattgctgcagctcagacccagtgctgccctggttgtggcttaggccaaagctgcagctccaattcaatctctggcctgggaacctccatgtgctacaaggtgcggccttaaaaggaaaaaaaaaaaattaaatcaaggactcaagagtctttcattatttgtgttgtggaagctatatttgttttaaagtcttagttgtgtttagaaagcaagatgttcttcaactcaaatttgggagggaacttgtttcatacatttttaatggataagtggcaaaattttcatgctgaggtgatctatagtgttgtaatgcagaatatagtcagatcttgaacattttaggaagttggtgagggccaattgtgtatctgtgccatgctgataagaatgtcaagggatcacaagaattcgtgttatttgacagcagtcatctttaaaaggcatttgagaaagtccaatttcaaatgcatttcctttctttaaaagataaattgaagaaaataagtctttatttcccaagtaaattgaattgcctctcagtctgttaaaagaaactcttaccttgatgattgcgctcttaacctggcaaagattgtctttaaaatctgagctccatgtcttctgctttatttctggtgtgcctttgactccagattacagtaaatggaggactgagtatagggctaaaaagtagagagaatggatgcatattatctgtggtctccaatgtgatgaatgaagtaggcaaatactcaaaggaaagagaaagcatgctccaagaattatgggttccagaaggcaaagtcccagaattgtctccagggaaggacagggaggtctagaatcggctaagcccactgtaggcagaaaaaccaagaggcatgaatggcttccctttctcacttttcactctctggcttactcctatcatgaaggaaaatattggaatcatattctccctcaccgaaatgctatttttcagcccacaggaaacccaggctggttggaggggacattccctgctctggtcgtgttgaagtacaacatggagacacgtggggcaccgtctgtgattctgacttctctctggaggcggccagcgtgctgtgcagggaactacagtgcggctactactactgtggtttccctcctggggggagctcactttggagaaggaagtggacagatctgggctgaagaattccagtgtgaggggcacgagtcccacctttcactctgcccagtagcaccccgccctgacgggacatgtagccacagcagggacgtcggcgtagtctgctcaagtgagacccagggaatgtgttcactttgttcccatgccatgaagagggtagggttaggtagtcacagacatctttttaaagccctgtctccttccaggatacacacaaatccgcttggtgaatggcaagaccccatgtgaaggaagagtggagctcaacattcttgggtcctgggggtccctctgcaactctcactgggacatggaagatgcccatgttttatgccagcagcttaaatgtggagttgccctttctatcccgggaggagcaccttttgggaaaggaagtgagcaggtctggaggcacatgtttcactgcactgggactgagaagcacatgggagattgttccgtcactgctctgggcgcatcactctgttcttcagggcaagtggcctctgtaatctgctcaggtaagagaataagggcagccagtgatgagccactcatgacggtgccttaagagtgggtgtacctaggagttcccattgtggctcagtggtaacaaactcgactggtatccatgagggtatgggtttgatccctggccttgctcaatgggttaaggatccagcattgctgtgagctgtggtataggttgcagactctgctcaggtcccatgttgctgtgattgtggtgtaggctgactgctgcagcttcaatttgacccctagcccgggaatttccataggccacacgtgcagcactaaggaaggaaaaaaagaaaaaaaaaaaaaaagagtgggtgtgcctatagtgaagaacagatgtaaaagggaagtgaaagggattcccccattctgagggattgtgagaagtgtgccagaatattaacttcatttgacttgttacagggaaagtaaacttgactttcacggacctcctagttacctggtgcttactatatgtcttctcagagtacctgattcattcccagcctggttgacccatccccctatctctatggctatgtttatccagagcacatctatctaacactccagctgatcttcctgacacagctgtggcaaccctggatcctttaaccaactgtgccaggctggagatcaaacctaagcctctgcagcaacccaagctgctgcagtcagatttttaaccccctgtgccactgtgggtatctccgatattttgtatcttctgtgactgagtggtttgctgtttgcagggaaccagagtcagacactatccccgtgcaattcatcatcctcggacccatcaagctctattatttcagaagaaaatggtgttgcctgcataggtgagaatcagtgaccaacctatgaaaatgatctcaatcctctgaaatgcattttattcatgttttatttcctctttgcagggagtggtcaacttcgcctggtcgatggaggtggtcgttgtgctgggagagtagaggtctatcatgagggctcctggggcaccatctgtgatgacagctgggacctgaatgatgcccatgtggtgtgcaaacagctgagctgtggatgggccattaatgccactggttctgctcattttggggaaggaacagggcccatttggctggatgagataaactgtaatggaaaagaatctcatatttggcaatgccactcacatggttgggggcggcacaattgcaggcataaggaggatgcaggagtcatctgctcgg

SEQ ID NO: 100 - DNA, 3710 bp, Sus scrofa
  source 1..3710: mol_type = other DNA
tatagatgacaaggctttgtgtctgataggggccagcgaactcagtaaagagggaagatgagaaagataatggcaagaatttatccctgaagtgtagttttgacaaaccagtcacaaagaggtctaagaaattttggtcacaaagttgttttgaatcccaggcattttatttgcaatgattgcatatgttctggaaaggacatctgaacctaagaaatagttcatttgcattgtgttatattttactaaggtctgagaaataatcttgagatgagaatgaactctacttcttcagagtctggaaggaataaattatgaaaatgtattaatgcttctttaaaccatattgtatatttatctattactaaacaaaaagaagtagctctatttatttatttatttatttatttatttatgtcttttgtctctttagggccacacctgtggcatatggaggttcccaggctagaggtccaattggagatgtagcagccagcctatgccagagccaccgcaacacgggatctgagccacgtctgtgacttacaccacagctcacagcaacgcctgatcctcaacccactgagcgaggccagggatcgaacccatgtcctcatggatgctagttgggttcgttaactgctgagccatgatgggaactccaaattaattatttcttatatttgttcttcatatattcatttctatagaaagaaataaatacagattcagttaatgatggcaggtaaaagcttaacttattaatcaaaggagttaatccaggcacaaaaattcaattcatggctctctgttaaaatttaggtataggtttagcaggaagaaaaggttagtagatgcagactattacatttagaatggatggacaatgaagtcctactatacagcacagggaactatatccaatctcttgggatagaatatgatggaagacaaaatcagaacaagagagtatatatatatgtgtgtgtgtgtgtgtgtgtgtgtgtgtgtgtgtgtgtgtgtgtgactgggtcaccctgcggcacagcagaaattggcagaacattgtaaatcaactatactttaataggaaaaatacttttaagggctaaatttccaatattctaaccatgtacacagagtaaatgtcataaggatgccagtctgtgtagagattgatgtgttactagcagattcatgaaataaaggctgaggatgtagtccccaagtcacttctgagtggaagaatttctcctttgtcctggactcaaatattttaggataaaggaaaaaagaagatatttatagaagggacttgttttcaagtacttgacaaaatttcaccattaaagagaaatttgtgggagttcccatcgtggctcagtggaaacaaatccaactaggaaccatgaggttgtgggtttgatccctggcctcactcagtgggttaaggatccggtgttgccgtgagctgtggtgtaggttgcagacacggttctgatcctgcgttgctgtggctgtggctgtggtgtaggccagcagcaaacagctctgattagacccctagcctggaaacctccatatgccacaggtgcagccctaaaaagacaaaaaaagagaaaagacaaaaaaaaaaaaaaaaaaaaaaaaaaaaaaaaaaaaaaaaaaaagaacccccagaggtatttatttgtttttgccttttttcactgactgttctttgtttgtttgtttgagactgatctagaagactagagattacaagaaatatggatttggctcactctaagaaactgctttcattccaaggtttgggtctatccaaaagtggaatagaatcatatgaatactagtttatgagtatttagtgagaggaatttcaagctcaaataatgattcagcaagattaaattaaggagggaattttccttgtggctgagtgggttaaggacccaatgttgtctctgtgaggatgtaggttccatcctgggctttgctcattaggttaaggatctggcattgctgcagctcagacccagtgctgccctggttgtggcttaggccaaagctgcagctccaattcaatctctggcctgggaacctccatgtgctacaaggtgcggccttaaaaggaaaaaaaaaaaattaaatcaaggactcaagagtctttcattatttgtgttgtggaagctatatttgttttaaagtcttagttgtgtttagaaagcaagatgttcttcaactcaaatttgggagggaacttgtttcatacatttttaatggataagtggcaaaattttcatgctgaggtgatctatagtgttgtaatgcagaatatagtcagatcttgaacattttaggaagttggtgagggccaattgtgtatctgtgccatgctgataagaatgtcaagggatcacaagaattcgtgttatttgacagcagtcatctttaaaaggcatttgagaaagtccaatttcaaatgcatttcctttctttaaaagataaattgaagaaaataagtctttatttcccaagtaaattgaattgcctctcagtctgttaaaagaaactcttaccttgatgattgcgctcttaacctggcaaagattgtctttaaaatctgagctccatgtcttctgctttatttctggtgtgcctttgactccagattacagtaaatggaggactgagtatagggctaaaaagtagagagaatggatgcatattatctgtggtctccaatgtgatgaatgaagtaggcaaatactcaaaggaaagagaaagcatgctccaagaattatgggttccagaagggaaagggattcccccattctgagggattgtgagaagtgtgccagaatattaacttcatttgacttgttacagggaaagtaaacttgactttcacggacctcctagttacctggtgcttactatatgtcttctcagagtacctgattcattcccagcctggttgacccatccccctatctctatggctatgtttatccagagcacatctatctaacactccagctgatcttcctgacacagctgtggcaaccctggatcctttaaccaactgtgccaggctggagatcaaacctaagcctctgcagcaacccaagctgctgcagtcagatttttaaccccctgtgccactgtgggtatctccgatattttgtatcttctgtgactgagtggtttgctgtttgcagggaaccagagtcagacactatccccgtgcaattcatcatcctcggacccatcaagctctattatttcagaagaaaatggtgttgcctgcataggtgagaatcagtgaccaacctatgaaaatgatctcaatcctctgaaatgcattttattcatgttttatttcctctttgcagggagtggtcaacttcgcctggtcgatggaggtggtcgttgtgctgggagagtagaggtctatcatgagggctcctggggcaccatctgtgatgacagctgggacctgaatgatgcccatgtggtgtgcaaacagctgagctgtggatgggccattaatgccactggttctgctcattttggggaaggaacagggcccatttggctggatgagataaactgtaatggaaaagaatctcatatttggcaatgccactcacatggttgggggcggcacaattgcaggcataaggaggatgcaggagtcatctgctcgg

SEQ ID NO: 101 - DNA, 3617 bp, Sus scrofa
  source 1..3617: mol_type = other DNA
tatagatgacaaggctttgtgtctgataggggccagcgaactcagtaaagagggaagatgagaaagataatggcaagaatttatccctgaagtgtagttttgacaaaccagtcacaaagaggtctaagaaattttggtcacaaagttgttttgaatcccaggcattttatttgcaatgattgcatatgttctggaaaggacatctgaacctaagaaatagttcatttgcattgtgttatattttactaaggtctgagaaataatcttgagatgagaatgaactctacttcttcagagtctggaaggaataaattatgaaaatgtattaatgcttctttaaaccatattgtatatttatctattactaaacaaaaagaagtagctctatttatttatttatttatttatttatttatgtcttttgtctctttagggccacacctgtggcatatggaggttcccaggctagaggtccaattggagatgtagcagccagcctatgccagagccaccgcaacacgggatctgagccacgtctgtgacttacaccacagctcacagcaacgcctgatcctcaacccactgagcgaggccagggatcgaacccatgtcctcatggatgctagttgggttcgttaactgctgagccatgatgggaactccaaattaattatttcttatatttgttcttcatatattcatttctatagaaagaaataaatacagattcagttaatgatggcaggtaaaagcttaacttattaatcaaaggagttaatccaggcacaaaaattcaattcatggctctctgttaaaatttaggtataggtttagcaggaagaaaaggttagtagatgcagactattacatttagaatggatggacaatgaagtcctactatacagcacagggaactatatccaatctcttgggatagaatatgatggaagacaaaatcagaacaagagagtatatatatatgtgtgtgtgtgtgtgtgtgtgtgtgtgtgtgtgtgtgtgtgtgtgactgggtcaccctgcggcacagcagaaattggcagaacattgtaaatcaactatactttaataggaaaaatacttttaagggctaaatttccaatattctaaccatgtacacagagtaaatgtcataaggatgccagtctgtgtagagattgatgtgttactagcagattcatgaaataaaggctgaggatgtagtccccaagtcacttctgagtggaagaatttctcctttgtcctggactcaaatattttaggataaaggaaaaaagaagatatttatagaagggacttgttttcaagtacttgacaaaatttcaccattaaagagaaatttgtgggagttcccatcgtggctcagtggaaacaaatccaactaggaaccatgaggttgtgggtttgatccctggcctcactcagtgggttaaggatccggtgttgccgtgagctgtggtgtaggttgcagacacggttctgatcctgcgttgctgtggctgtggctgtggtgtaggccagcagcaaacagctctgattagacccctagcctggaaacctccatatgccacaggtgcagccctaaaaagacaaaaaaagagaaaagacaaaaaaaaaaaaaaaaaaaaaaaaaaaaaaaaaaaaaaaaaaaagaacccccagaggtatttatttgtttttgccttttttcactgactgttctttgtttgtttgtttgagactgatctagaagactagagattacaagaaatatggatttggctcactctaagaaactgctttcattccaaggtttgggtctatccaaaagtggaatagaatcatatgaatactagtttatgagtatttagtgagaggaatttcaagctcaaataatgattcagcaagattaaattaaggagggaattttccttgtggctgagtgggttaaggacccaatgttgtctctgtgaggatgtaggttccatcctgggctttgctcattaggttaaggatctggcattgctgcagctcagacccagtgctgccctggttgtggcttaggccaaagctgcagctccaattcaatctctggcctgggaacctccatgtgctacaaggtgcggccttaaaaggaaaaaaaaaaaattaaatcaaggactcaagagtctttcattatttgtgttgtggaagctatatttgttttaaagtcttagttgtgtttagaaagcaagatgttcttcaactcaaatttgggagggaacttgtttcatacatttttaatggataagtggcaaaattttcatgctgaggtgatctatagtgttgtaatgcagaatatagtcagatcttgaacattttaggaagttggtgagggccaattgtgtatctgtgccatgctgataagaatgtcaagggatcacaagaattcgtgttatttgacagcagtcatctttaaaaggcatttgagaaagtccaatttcaaatgcatttcctttctttaaaagataaattgaagaaaataagtctttatttcccaagtaaattgaattgcctctcagtctgttaaaagaaactcttaccttgatgattgcgctcttaacctggcaaagattgtctttaaaatctgagctccatgtcttctgctttatttctggtgtgcctttgactccagattacagtaaatggaggactgagtatagggctaaaaagtagagagaatggattgaaagggattcccccattctgagggattgtgagaagtgtgccagaatattaacttcatttgacttgttacagggaaagtaaacttgactttcacggacctcctagttacctggtgcttactatatgtcttctcagagtacctgattcattcccagcctggttgacccatccccctatctctatggctatgtttatccagagcacatctatctaacactccagctgatcttcctgacacagctgtggcaaccctggatcctttaaccaactgtgccaggctggagatcaaacctaagcctctgcagcaacccaagctgctgcagtcagatttttaaccccctgtgccactgtgggtatctccgatattttgtatcttctgtgactgagtggtttgctgtttgcagggaaccagagtcagacactatccccgtgcaattcatcatcctcggacccatcaagctctattatttcagaagaaaatggtgttgcctgcataggtgagaatcagtgaccaacctatgaaaatgatctcaatcctctgaaatgcattttattcatgttttatttcctctttgcagggagtggtcaacttcgcctggtcgatggaggtggtcgttgtgctgggagagtagaggtctatcatgagggctcctggggcaccatctgtgatgacagctgggacctgaatgatgcccatgtggtgtgcaaacagctgagctgtggatgggccattaatgccactggttctgctcattttggggaaggaacagggcccatttggctggatgagataaactgtaatggaaaagaatctcatatttggcaatgccactcacatggttgggggcggcacaattgcaggcataaggaggatgcaggagtcatctgctcgg

SEQ ID NO: 102 - DNA, 4979 bp, Sus scrofa
  source 1..4979: mol_type = other DNA
tatagatgacaaggctttgtgtctgataggggccagcgaactcagtaaagagggaagatgagaaagataatggcaagaatttatccctgaagtgtagttttgacaaaccagtcacaaagaggtctaagaaattttggtcacaaagttgttttgaatcccaggcattttatttgcaatgattgcatatgttctggaaaggacatctgaacctaagaaatagttcatttgcattgtgttatattttactaaggtctgagaaataatcttgagatgagaatgaactctacttcttcagagtctggaaggaataaattatgaaaatgtattaatgcttctttaaaccatattgtatatttatctattactaaacaaaaagaagtagctctatttatttatttatttatttatttatttatgtcttttgtctctttagggccacacctgtggcatatggaggttcccaggctagaggtccaattggagatgtagcagccagcctatgccagagccaccgcaacacgggatctgagccacgtctgtgacttacaccacagctcacagcaacgcctgatcctcaacccactgagcgaggccagggatcgaacccatgtcctcatggatgctagttgggttcgttaactgctgagccatgatgggaactccaaattaattatttcttatatttgttcttcatatattcatttctatagaaagaaataaatacagattcagttaatgatggcaggtaaaagcttaacttattaatcaaaggagttaatccaggcacaaaaattcaattcatggctctctgttaaaatttaggtataggtttagcaggaagaaaaggttagtagatgcagactattacatttagaatggatggacaatgaagtcctactatacagcacagggaactatatccaatctcttgggatagaatatgatggaagacaaaatcagaacaagagagtatatatatatgtgtgtgtgtgtgtgtgtgtgtgtgtgtgtgtgtgtgtgtgtgtgactgggtcaccctgcggcacagcagaaattggcagaacattgtaaatcaactatactttaataggaaaaatacttttaagggctaaatttccaatattctaaccatgtacacagagtaaatgtcataaggatgccagtctgtgtagagattgatgtgttactagcagattcatgaaataaaggctgaggatgtagtccccaagtcacttctgagtggaagaatttctcctttgtcctggactcaaatattttaggataaaggaaaaaagaagatatttatagaagggacttgttttcaagtacttgacaaaatttcaccattaaagagaaatttgtgggagttcccatcgtggctcagtggaaacaaatccaactaggaaccatgaggttgtgggtttgatccctggcctcactcagtgggttaaggatccggtgttgccgtgagctgtggtgtaggttgcagacacggttctgatcctgcgttgctgtggctgtggctgtggtgtaggccagcagcaaacagctctgattagacccctagcctggaaacctccatatgccacaggtgcagccctaaaaagacaaaaaaagagaaaagacaaaaaaaaaaaaaaaaaaaaaaaaaaaaaaaaaaaaaaaaaaaagaacccccagaggtatttatttgtttttgccttttttcactgactgttctttgtttgtttgtttgagactgatctagaagactagagattacaagaaatatggatttggctcactctaagaaactgctttcattccaaggtttgggtctatccaaaagtggaatagaatcatatgaatactagtttatgagtatttagtgagaggaatttcaagctcaaataatgattcagcaagattaaattaaggagggaattttccttgtggctgagtgggttaaggacccaatgttgtctctgtgaggatgtaggttccatcctgggctttgctcattaggttaaggatctggcattgctgcagctcagacccagtgctgccctggttgtggcttaggccaaagctgcagctccaattcaatctctggcctgggaacctccatgtgctacaaggtgcggccttaaaaggaaaaaaaaaaaattaaatcaaggactcaagagtctttcattatttgtgttgtggaagctatatttgttttaaagtcttagttgtgtttagaaagcaagatgttcttcaactcaaatttgggagggaacttgtttcatacatttttaatggataagtggcaaaattttcatgctgaggtgatctatagtgttgtaatgcagaatatagtcagatcttgaacattttaggaagttggtgagggccaattgtgtatctgtgccatgctgataagaatgtcaagggatcacaagaattcgtgttatttgacagcagtcatctttaaaaggcatttgagaaagtccaatttcaaatgcatttcctttctttaaaagataaattgaagaaaataagtctttatttcccaagtaaattgaattgcctctcagtctgttaaaagaaactcttaccttgatgattgcgctcttaacctggcaaagattgtctttaaaatctgagctccatgtcttctgctttatttctggtgtgcctttgactccagattacagtaaatggaggactgagtatagggctaaaaagtagagagaatggatgcatattatctgtggtctccaatgtgatgaatgaagtaggcaaatactcaaaggaaagagaaagcatgctccaagaattatgggttccagaaggcaaagtcccagaattgtctccagggaaggacagggaggtctagaatcggctaagcccactgtaggcagaaaaaccaagaggcatgaatggcttccctttctcacttttcactctctggcttactcctatcatgaaggaaaatattggaatcatattctccctcaccgaaatgctatttttcagcccacaggaaacccaggctggttggaggggacattccctgctctggtcgtgttgaagtacaacatggagacacgtggggcaccgtctgtgattctgacttctctctggaggcggccagcgtgctgtgcagggaactctgtggtttccctcctggggggagctcactttggagaaggaagtggacagatctgggctgaagaattccagtgtgaggggcacgagtcccacctttcactctgcccagtagcaccccgccctgacgggacatgtagccacagcagggacgtcggcgtagtctgctcaagtgagacccagggaatgtgttcactttgttcccatgccatgaagagggtagggttaggtagtcacagacatctttttaaagccctgtctccttccaggatacacacaaatccgcttggtgaatggcaagaccccatgtgaaggaagagtggagctcaacattcttgggtcctgggggtccctctgcaactctcactgggacatggaagatgcccatgttttatgccagcagcttaaatgtggagttgccctttctatcccgggaggagcaccttttgggaaaggaagtgagcaggtctggaggcacatgtttcactgcactgggactgagaagcacatgggagattgttccgtcactgctctgggcgcatcactctgttcttcagggcaagtggcctctgtaatctgctcaggtaagagaataagggcagccagtgatgagccactcatgacggtgccttaagagtgggtgtacctaggagttcccattgtggctcagtggtaacaaactcgactggtatccatgagggtatgggtttgatccctggccttgctcaatgggttaaggatccagcattgctgtgagctgtggtataggttgcagactctgctcaggtcccatgttgctgtgattgtggtgtaggctgactgctgcagcttcaatttgacccctagcccgggaatttccataggccacacgtgcagcactaaggaaggaaaaaaagaaaaaaaaaaaaaaagagtgggtgtgcctatagtgaagaacagatgtaaaagggaagtgaaagggattcccccattctgagggattgtgagaagtgtgccagaatattaacttcatttgacttgttacagggaaagtaaacttgactttcacggacctcctagttacctggtgcttactatatgtcttctcagagtacctgattcattcccagcctggttgacccatccccctatctctatggctatgtttatccagagcacatctatctaacactccagctgatcttcctgacacagctgtggcaaccctggatcctttaaccaactgtgccaggctggagatcaaacctaagcctctgcagcaacccaagctgctgcagtcagatttttaaccccctgtgccactgtgggtatctccgatattttgtatcttctgtgactgagtggtttgctgtttgcagggaaccagagtcagacactatccccgtgcaattcatcatcctcggacccatcaagctctattatttcagaagaaaatggtgttgcctgcataggtgagaatcagtgaccaacctatgaaaatgatctcaatcctctgaaatgcattttattcatgttttatttcctctttgcagggagtggtcaacttcgcctggtcgatggaggtggtcgttgtgctgggagagtagaggtctatcatgagggctcctggggcaccatctgtgatgacagctgggacctgaatgatgcccatgtggtgtgcaaacagctgagctgtggatgggccattaatgccactggttctgctcattttggggaaggaacagggcccatttggctggatgagataaactgtaatggaaaagaatctcatatttggcaatgccactcacatggttgggggcggcacaattgcaggcataaggaggatgcaggagtcatctgctcgg

SEQ ID NO: 103 - DNA, 4615 bp, Sus scrofa
  source 1..4615: mol_type = other DNA
tatagatgacaaggctttgtgtctgataggggccagcgaactcagtaaagagggaagatgagaaagataatggcaagaatttatccctgaagtgtagttttgacaaaccagtcacaaagaggtctaagaaattttggtcacaaagttgttttgaatcccaggcattttatttgcaatgattgcatatgttctggaaaggacatctgaacctaagaaatagttcatttgcattgtgttatattttactaaggtctgagaaataatcttgagatgagaatgaactctacttcttcagagtctggaaggaataaattatgaaaatgtattaatgcttctttaaaccatattgtatatttatctattactaaacaaaaagaagtagctctatttatttatttatttatttatttatttatgtcttttgtctctttagggccacacctgtggcatatggaggttcccaggctagaggtccaattggagatgtagcagccagcctatgccagagccaccgcaacacgggatctgagccacgtctgtgacttacaccacagctcacagcaacgcctgatcctcaacccactgagcgaggccagggatcgaacccatgtcctcatggatgctagttgggttcgttaactgctgagccatgatgggaactccaaattaattatttcttatatttgttcttcatatattcatttctatagaaagaaataaatacagattcagttaatgatggcaggtaaaagcttaacttattaatcaaaggagttaatccaggcacaaaaattcaattcatggctctctgttaaaatttaggtataggtttagcaggaagaaaaggttagtagatgcagactattacatttagaatggatggacaatgaagtcctactatacagcacagggaactatatccaatctcttgggatagaatatgatggaagacaaaatcagaacaagagagtatatatatatgtgtgtgtgtgtgtgtgtgtgtgtgtgtgtgtgtgtgtgtgtgtgactgggtcaccctgcggcacagcagaaattggcagaacattgtaaatcaactatactttaataggaaaaatacttttaagggctaaatttccaatattctaaccatgtacacagagtaaatgtcataaggatgccagtctgtgtagagattgatgtgttactagcagattcatgaaataaaggctgaggatgtagtccccaagtcacttctgagtggaagaatttctcctttgtcctggactcaaatattttaggataaaggaaaaaagaagatatttatagaagggacttgttttcaagtacttgacaaaatttcaccattaaagagaaatttgtgggagttcccatcgtggctcagtggaaacaaatccaactaggaaccatgaggttgtgggtttgatccctggcctcactcagtgggttaaggatccggtgttgccgtgagctgtggtgtaggttgcagacacggttctgatcctgcgttgctgtggctgtggctgtggtgtaggccagcagcaaacagctctgattagacccctagcctggaaacctccatatgccacaggtgcagccctaaaaagacaaaaaaagagaaaagacaaaaaaaaaaaaaaaaaaaaaaaaaaaaaaaaaaaaaaaaaaaagaacccccagaggtatttatttgtttttgccttttttcactgactgttctttgtttgtttgtttgagactgatctagaagactagagattacaagaaatatggatttggctcactctaagaaactgctttcattccaaggtttgggtctatccaaaagtggaatagaatcatatgaatactagtttatgagtatttagtgagaggaatttcaagctcaaataatgattcagcaagattaaattaaggagggaattttccttgtggctgagtgggttaaggacccaatgttgtctctgtgaggatgtaggttccatcctgggctttgctcattaggttaaggatctggcattgctgcagctcagacccagtgctgccctggttgtggcttaggccaaagctgcagctccaattcaatctctggcctgggaacctccatgtgctacaaggtgcggccttaaaaggaaaaaaaaaaaattaaatcaaggactcaagagtctttcattatttgtgttgtggaagctatatttgttttaaagtcttagttgtgtttagaaagcaagatgttcttcaactcaaatttgggagggaacttgtttcatacatttttaatggataagtggcaaaattttcatgctgaggtgatctatagtgttgtaatgcagaatatagtcagatcttgaacattttaggaagttggtgagggccaattgtgtatctgtgccatgctgataagaatgtcaagggatcacaagaattcgtgttatttgacagcagtcatctttaaaaggcatttgagaaagtccaatttcaaatgcatttcctttctttaaaagataaattgaagaaaataagtctttatttcccaagtaaattgaattgcctctcagtctgttaaaagaaagaaggaaaatattggaatcatattctccctcaccgaaatgctatttttcagcccacaggaaacccaggctggttggaggggacattccctgctctggtcgtgttgaagtacaacatggagacacgtggggcaccgtctgtgattctgacttctctctggaggcggccagcgtgctgtgcagggaactacagtgcggcacagtgtggtttccctcctggggggagctcactttggagaaggaagtggacagatctgggctgaagaattccagtgtgaggggcacgagtcccacctttcactctgcccagtagcaccccgccctgacgggacatgtagccacagcagggacgtcggcgtagtctgctcaagtgagacccagggaatgtgttcactttgttcccatgccatgaagagggtagggttaggtagtcacagacatctttttaaagccctgtctccttccaggatacacacaaatccgcttggtgaatggcaagaccccatgtgaaggaagagtggagctcaacattcttgggtcctgggggtccctctgcaactctcactgggacatggaagatgcccatgttttatgccagcagcttaaatgtggagttgccctttctatcccgggaggagcaccttttgggaaaggaagtgagcaggtctggaggcacatgtttcactgcactgggactgagaagcacatgggagattgttccgtcactgctctgggcgcatcactctgttcttcagggcaagtggcctctgtaatctgctcaggtaagagaataagggcagccagtgatgagccactcatgacggtgccttaagagtgggtgtacctaggagttcccattgtggctcagtggtaacaaactcgactggtatccatgagggtatgggtttgatccctggccttgctcaatgggttaaggatccagcattgctgtgagctgtggtataggttgcagactctgctcaggtcccatgttgctgtgattgtggtgtaggctgactgctgcagcttcaatttgacccctagcccgggaatttccataggccacacgtgcagcactaaggaaggaaaaaaagaaaaaaaaaaaaaaagagtgggtgtgcctatagtgaagaacagatgtaaaagggaagtgaaagggattcccccattctgagggattgtgagaagtgtgccagaatattaacttcatttgacttgttacagggaaagtaaacttgactttcacggacctcctagttacctggtgcttactatatgtcttctcagagtacctgattcattcccagcctggttgacccatccccctatctctatggctatgtttatccagagcacatctatctaacactccagctgatcttcctgacacagctgtggcaaccctggatcctttaaccaactgtgccaggctggagatcaaacctaagcctctgcagcaacccaagctgctgcagtcagatttttaaccccctgtgccactgtgggtatctccgatattttgtatcttctgtgactgagtggtttgctgtttgcagggaaccagagtcagacactatccccgtgcaattcatcatcctcggacccatcaagctctattatttcagaagaaaatggtgttgcctgcataggtgagaatcagtgaccaacctatgaaaatgatctcaatcctctgaaatgcattttattcatgttttatttcctctttgcagggagtggtcaacttcgcctggtcgatggaggtggtcgttgtgctgggagagtagaggtctatcatgagggctcctggggcaccatctgtgatgacagctgggacctgaatgatgcccatgtggtgtgcaaacagctgagctgtggatgggccattaatgccactggttctgctcattttggggaaggaacagggcccatttggctggatgagataaactgtaatggaaaagaatctcatatttggcaatgccactcacatggttgggggcggcacaattgcaggcataaggaggatgcaggagtcatctgctcgg

SEQ ID NO: 104 - DNA, 4866 bp, Sus scrofa
  source 1..4866: mol_type = other DNA
tatagatgacaaggctttgtgtctgataggggccagcgaactcagtaaagagggaagatgagaaagataatggcaagaatttatccctgaagtgtagttttgacaaaccagtcacaaagaggtctaagaaattttggtcacaaagttgttttgaatcccaggcattttatttgcaatgattgcatatgttctggaaaggacatctgaacctaagaaatagttcatttgcattgtgttatattttactaaggtctgagaaataatcttgagatgagaatgaactctacttcttcagagtctggaaggaataaattatgaaaatgtattaatgcttctttaaaccatattgtatatttatctattactaaacaaaaagaagtagctctatttatttatttatttatttatttatttatgtcttttgtctctttagggccacacctgtggcatatggaggttcccaggctagaggtccaattggagatgtagcagccagcctatgccagagccaccgcaacacgggatctgagccacgtctgtgacttacaccacagctcacagcaacgcctgatcctcaacccactgagcgaggccagggatcgaacccatgtcctcatggatgctagttgggttcgttaactgctgagccatgatgggaactccaaattaattatttcttatatttgttcttcatatattcatttctatagaaagaaataaatacagattcagttaatgatggcaggtaaaagcttaacttattaatcaaaggagttaatccaggcacaaaaattcaattcatggctctctgttaaaatttaggtataggtttagcaggaagaaaaggttagtagatgcagactattacatttagaatggatggacaatgaagtcctactatacagcacagggaactatatccaatctcttgggatagaatatgatggaagacaaaatcagaacaagagagtatatatatatgtgtgtgtgtgtgtgtgtgtgtgtgtgtgtgtgtgtgtgtgtgtgactgggtcaccctgcggcacagcagaaattggcagaacattgtaaatcaactatactttaataggaaaaatacttttaagggctaaatttccaatattctaaccatgtacacagagtaaatgtcataaggatgccagtctgtgtagagattgatgtgttactagcagattcatgaaataaaggctgaggatgtagtccccaagtcacttctgagtggaagaatttctcctttgtcctggactcaaatattttaggataaaggaaaaaagaagatatttatagaagggacttgttttcaagtacttgacaaaatttcaccattaaagagaaatttgtgggagttcccatcgtggctcagtggaaacaaatccaactaggaaccatgaggttgtgggtttgatccctggcctcactcagtgggttaaggatccggtgttgccgtgagctgtggtgtaggttgcagacacggttctgatcctgcgttgctgtggctgtggctgtggtgtaggccagcagcaaacagctctgattagacccctagcctggaaacctccatatgccacaggtgcagccctaaaaagacaaaaaaagagaaaagacaaaaaaaaaaaaaaaaaaaaaaaaaaaaaaaaaaaaaaaaaaaagaacccccagaggtatttatttgtttttgccttttttcactgactgttctttgtttgtttgtttgagactgatctagaagactagagattacaagaaatatggatttggctcactctaagaaactgctttcattccaaggtttgggtctatccaaaagtggaatagaatcatatgaatactagtttatgagtatttagtgagaggaatttcaagctcaaataatgattcagcaagattaaattaaggagggaattttccttgtggctgagtgggttaaggacccaatgttgtctctgtgaggatgtaggttccatcctgggctttgctcattaggttaaggatctggcattgctgcagctcagacccagtgctgccctggttgtggcttaggccaaagctgcagctccaattcaatctctggcctgggaacctccatgtgctacaaggtgcggccttaaaaggaaaaaaaaaaaattaaatcaaggactcaagagtctttcattatttgtgttgtggaagctatatttgttttaaagtcttagttgtgtttagaaagcaagatgttcttcaactcaaatttgggagggaacttgtttcatacatttttaatggataagtggcaaaattttcatgctgaggtgatctatagtgttgtaatgcagaatatagtcagatcttgaacattttaggaagttggtgagggccaattgtgtatctgtgccatgctgataagaatgtcaagggatcacaagaattcgtgttatttgacagcagtcatctttaaaaggcatttgagaaagtccaatttcaaatgcatttcctttctttaaaagataaattgaagaaaataagtctttatttcccaagtaaattgaattgcctctcagtctgttaaaagaaactcttaccttgatgattgcgctcttaacctggcaaagattgtctttaaaatctgagctccatgtcttctgctttatttctggtgtgcctttgactccagattacagtaaatggaggactgagtatagggctaaaaagtagagagaatggatgcatattatctgtggtctccaatgtgatgaatgaagtaggcaaatactcaaaggaaagagaaagcatgctccaagaattatgggttccagaaggcaaagtcccagaattgtctccagggaaggacagggaggtctagaatcggctaagcccactgtaggcagaaaaaccaagaggcatgaatggcttccctttctcacttttcactctctggcttactcctatcatgaaggaaaatattggaatcatattctccctcaccgaaatgctatttttcagcccacaggaaacccaggctggttctgtggtttccctcctggggggagctcactttggagaaggaagtggacagatctgggctgaagaattccagtgtgaggggcacgagtcccacctttcactctgcccagtagcaccccgccctgacgggacatgtagccacagcagggacgtcggcgtagtctgctcaagtgagacccagggaatgtgttcactttgttcccatgccatgaagagggtagggttaggtagtcacagacatctttttaaagccctgtctccttccaggatacacacaaatccgcttggtgaatggcaagaccccatgtgaaggaagagtggagctcaacattcttgggtcctgggggtccctctgcaactctcactgggacatggaagatgcccatgttttatgccagcagcttaaatgtggagttgccctttctatcccgggaggagcaccttttgggaaaggaagtgagcaggtctggaggcacatgtttcactgcactgggactgagaagcacatgggagattgttccgtcactgctctgggcgcatcactctgttcttcagggcaagtggcctctgtaatctgctcaggtaagagaataagggcagccagtgatgagccactcatgacggtgccttaagagtgggtgtacctaggagttcccattgtggctcagtggtaacaaactcgactggtatccatgagggtatgggtttgatccctggccttgctcaatgggttaaggatccagcattgctgtgagctgtggtataggttgcagactctgctcaggtcccatgttgctgtgattgtggtgtaggctgactgctgcagcttcaatttgacccctagcccgggaatttccataggccacacgtgcagcactaaggaaggaaaaaaagaaaaaaaaaaaaaaagagtgggtgtgcctatagtgaagaacagatgtaaaagggaagtgaaagggattcccccattctgagggattgtgagaagtgtgccagaatattaacttcatttgacttgttacagggaaagtaaacttgactttcacggacctcctagttacctggtgcttactatatgtcttctcagagtacctgattcattcccagcctggttgacccatccccctatctctatggctatgtttatccagagcacatctatctaacactccagctgatcttcctgacacagctgtggcaaccctggatcctttaaccaactgtgccaggctggagatcaaacctaagcctctgcagcaacccaagctgctgcagtcagatttttaaccccctgtgccactgtgggtatctccgatattttgtatcttctgtgactgagtggtttgctgtttgcagggaaccagagtcagacactatccccgtgcaattcatcatcctcggacccatcaagctctattatttcagaagaaaatggtgttgcctgcataggtgagaatcagtgaccaacctatgaaaatgatctcaatcctctgaaatgcattttattcatgttttatttcctctttgcagggagtggtcaacttcgcctggtcgatggaggtggtcgttgtgctgggagagtagaggtctatcatgagggctcctggggcaccatctgtgatgacagctgggacctgaatgatgcccatgtggtgtgcaaacagctgagctgtggatgggccattaatgccactggttctgctcattttggggaaggaacagggcccatttggctggatgagataaactgtaatggaaaagaatctcatatttggcaatgccactcacatggttgggggcggcacaattgcaggcataaggaggatgcaggagtcatctgctcgg

SEQ ID NO: 105 - DNA, 4867 bp, Sus scrofa
  source 1..4867: mol_type = other DNA
tatagatgacaaggctttgtgtctgataggggccagcgaactcagtaaagagggaagatgagaaagataatggcaagaatttatccctgaagtgtagttttgacaaaccagtcacaaagaggtctaagaaattttggtcacaaagttgttttgaatcccaggcattttatttgcaatgattgcatatgttctggaaaggacatctgaacctaagaaatagttcatttgcattgtgttatattttactaaggtctgagaaataatcttgagatgagaatgaactctacttcttcagagtctggaaggaataaattatgaaaatgtattaatgcttctttaaaccatattgtatatttatctattactaaacaaaaagaagtagctctatttatttatttatttatttatttatttatgtcttttgtctctttagggccacacctgtggcatatggaggttcccaggctagaggtccaattggagatgtagcagccagcctatgccagagccaccgcaacacgggatctgagccacgtctgtgacttacaccacagctcacagcaacgcctgatcctcaacccactgagcgaggccagggatcgaacccatgtcctcatggatgctagttgggttcgttaactgctgagccatgatgggaactccaaattaattatttcttatatttgttcttcatatattcatttctatagaaagaaataaatacagattcagttaatgatggcaggtaaaagcttaacttattaatcaaaggagttaatccaggcacaaaaattcaattcatggctctctgttaaaatttaggtataggtttagcaggaagaaaaggttagtagatgcagactattacatttagaatggatggacaatgaagtcctactatacagcacagggaactatatccaatctcttgggatagaatatgatggaagacaaaatcagaacaagagagtatatatatatgtgtgtgtgtgtgtgtgtgtgtgtgtgtgtgtgtgtgtgtgtgtgactgggtcaccctgcggcacagcagaaattggcagaacattgtaaatcaactatactttaataggaaaaatacttttaagggctaaatttccaatattctaaccatgtacacagagtaaatgtcataaggatgccagtctgtgtagagattgatgtgttactagcagattcatgaaataaaggctgaggatgtagtccccaagtcacttctgagtggaagaatttctcctttgtcctggactcaaatattttaggataaaggaaaaaagaagatatttatagaagggacttgttttcaagtacttgacaaaatttcaccattaaagagaaatttgtgggagttcccatcgtggctcagtggaaacaaatccaactaggaaccatgaggttgtgggtttgatccctggcctcactcagtgggttaaggatccggtgttgccgtgagctgtggtgtaggttgcagacacggttctgatcctgcgttgctgtggctgtggctgtggtgtaggccagcagcaaacagctctgattagacccctagcctggaaacctccatatgccacaggtgcagccctaaaaagacaaaaaaagagaaaagacaaaaaaaaaaaaaaaaaaaaaaaaaaaaaaaaaaaaaaaaaaaagaacccccagaggtatttatttgtttttgccttttttcactgactgttctttgtttgtttgtttgagactgatctagaagactagagattacaagaaatatggatttggctcactctaagaaactgctttcattccaaggtttgggtctatccaaaagtggaatagaatcatatgaatactagtttatgagtatttagtgagaggaatttcaagctcaaataatgattcagcaagattaaattaaggagggaattttccttgtggctgagtgggttaaggacccaatgttgtctctgtgaggatgtaggttccatcctgggctttgctcattaggttaaggatctggcattgctgcagctcagacccagtgctgccctggttgtggcttaggccaaagctgcagctccaattcaatctctggcctgggaacctccatgtgctacaaggtgcggccttaaaaggaaaaaaaaaaaattaaatcaaggactcaagagtctttcattatttgtgttgtggaagctatatttgttttaaagtcttagttgtgtttagaaagcaagatgttcttcaactcaaatttgggagggaacttgtttcatacatttttaatggataagtggcaaaattttcatgctgaggtgatctatagtgttgtaatgcagaatatagtcagatcttgaacattttaggaagttggtgagggccaattgtgtatctgtgccatgctgataagaatgtcaagggatcacaagaattcgtgttatttgacagcagtcatctttaaaaggcatttgagaaagtccaatttcaaatgcatttcctttctttaaaagataaattgaagaaaataagtctttatttcccaagtaaattgaattgcctctcagtctgttaaaagaaactcttaccttgatgattgcgctcttaacctggcaaagattgtctttaaaatctgagctccatgtcttctgctttatttctggtgtgcctttgactccagattacagtaaatggaggactgagtatagggctaaaaagtagagagaatggatgcatattatctgtggtctccaatgtgatgaatgaagtaggcaaatactcaaaggaaagagaaagcatgctccaagaattatgggttccagaaggcaaagtcccagaattgtctccagggaaggacagggaggtctagaatcggctaagcccactgtaggcagaaaaaccaagaggcatgaatggcttccctttctcacttttcactctctggcttactcctatcatgaaggaaaatattggaatcatattctccctcaccgaaatgctatttttcagcccacaggaaacccaggctggttactgtggtttccctcctggggggagctcactttggagaaggaagtggacagatctgggctgaagaattccagtgtgaggggcacgagtcccacctttcactctgcccagtagcaccccgccctgacgggacatgtagccacagcagggacgtcggcgtagtctgctcaagtgagacccagggaatgtgttcactttgttcccatgccatgaagagggtagggttaggtagtcacagacatctttttaaagccctgtctccttccaggatacacacaaatccgcttggtgaatggcaagaccccatgtgaaggaagagtggagctcaacattcttgggtcctgggggtccctctgcaactctcactgggacatggaagatgcccatgttttatgccagcagcttaaatgtggagttgccctttctatcccgggaggagcaccttttgggaaaggaagtgagcaggtctggaggcacatgtttcactgcactgggactgagaagcacatgggagattgttccgtcactgctctgggcgcatcactctgttcttcagggcaagtggcctctgtaatctgctcaggtaagagaataagggcagccagtgatgagccactcatgacggtgccttaagagtgggtgtacctaggagttcccattgtggctcagtggtaacaaactcgactggtatccatgagggtatgggtttgatccctggccttgctcaatgggttaaggatccagcattgctgtgagctgtggtataggttgcagactctgctcaggtcccatgttgctgtgattgtggtgtaggctgactgctgcagcttcaatttgacccctagcccgggaatttccataggccacacgtgcagcactaaggaaggaaaaaaagaaaaaaaaaaaaaaagagtgggtgtgcctatagtgaagaacagatgtaaaagggaagtgaaagggattcccccattctgagggattgtgagaagtgtgccagaatattaacttcatttgacttgttacagggaaagtaaacttgactttcacggacctcctagttacctggtgcttactatatgtcttctcagagtacctgattcattcccagcctggttgacccatccccctatctctatggctatgtttatccagagcacatctatctaacactccagctgatcttcctgacacagctgtggcaaccctggatcctttaaccaactgtgccaggctggagatcaaacctaagcctctgcagcaacccaagctgctgcagtcagatttttaaccccctgtgccactgtgggtatctccgatattttgtatcttctgtgactgagtggtttgctgtttgcagggaaccagagtcagacactatccccgtgcaattcatcatcctcggacccatcaagctctattatttcagaagaaaatggtgttgcctgcataggtgagaatcagtgaccaacctatgaaaatgatctcaatcctctgaaatgcattttattcatgttttatttcctctttgcagggagtggtcaacttcgcctggtcgatggaggtggtcgttgtgctgggagagtagaggtctatcatgagggctcctggggcaccatctgtgatgacagctgggacctgaatgatgcccatgtggtgtgcaaacagctgagctgtggatgggccattaatgccactggttctgctcattttggggaaggaacagggcccatttggctggatgagataaactgtaatggaaaagaatctcatatttggcaatgccactcacatggttgggggcggcacaattgcaggcataaggaggatgcaggagtcatctgctcgg

SEQ ID NO: 106 - DNA, 4991 bp, Sus scrofa
  source 1..4991: mol_type = other DNA
tatagatgacaaggctttgtgtctgataggggccagcgaactcagtaaagagggaagatgagaaagataatggcaagaatttatccctgaagtgtagttttgacaaaccagtcacaaagaggtctaagaaattttggtcacaaagttgttttgaatcccaggcattttatttgcaatgattgcatatgttctggaaaggacatctgaacctaagaaatagttcatttgcattgtgttatattttactaaggtctgagaaataatcttgagatgagaatgaactctacttcttcagagtctggaaggaataaattatgaaaatgtattaatgcttctttaaaccatattgtatatttatctattactaaacaaaaagaagtagctctatttatttatttatttatttatttatttatgtcttttgtctctttagggccacacctgtggcatatggaggttcccaggctagaggtccaattggagatgtagcagccagcctatgccagagccaccgcaacacgggatctgagccacgtctgtgacttacaccacagctcacagcaacgcctgatcctcaacccactgagcgaggccagggatcgaacccatgtcctcatggatgctagttgggttcgttaactgctgagccatgatgggaactccaaattaattatttcttatatttgttcttcatatattcatttctatagaaagaaataaatacagattcagttaatgatggcaggtaaaagcttaacttattaatcaaaggagttaatccaggcacaaaaattcaattcatggctctctgttaaaatttaggtataggtttagcaggaagaaaaggttagtagatgcagactattacatttagaatggatggacaatgaagtcctactatacagcacagggaactatatccaatctcttgggatagaatatgatggaagacaaaatcagaacaagagagtatatatatatgtgtgtgtgtgtgtgtgtgtgtgtgtgtgtgtgtgtgtgtgtgtgactgggtcaccctgcggcacagcagaaattggcagaacattgtaaatcaactatactttaataggaaaaatacttttaagggctaaatttccaatattctaaccatgtacacagagtaaatgtcataaggatgccagtctgtgtagagattgatgtgttactagcagattcatgaaataaaggctgaggatgtagtccccaagtcacttctgagtggaagaatttctcctttgtcctggactcaaatattttaggataaaggaaaaaagaagatatttatagaagggacttgttttcaagtacttgacaaaatttcaccattaaagagaaatttgtgggagttcccatcgtggctcagtggaaacaaatccaactaggaaccatgaggttgtgggtttgatccctggcctcactcagtgggttaaggatccggtgttgccgtgagctgtggtgtaggttgcagacacggttctgatcctgcgttgctgtggctgtggctgtggtgtaggccagcagcaaacagctctgattagacccctagcctggaaacctccatatgccacaggtgcagccctaaaaagacaaaaaaagagaaaagacaaaaaaaaaaaaaaaaaaaaaaaaaaaaaaaaaaaaaaaaaaaagaacccccagaggtatttatttgtttttgccttttttcactgactgttctttgtttgtttgtttgagactgatctagaagactagagattacaagaaatatggatttggctcactctaagaaactgctttcattccaaggtttgggtctatccaaaagtggaatagaatcatatgaatactagtttatgagtatttagtgagaggaatttcaagctcaaataatgattcagcaagattaaattaaggagggaattttccttgtggctgagtgggttaaggacccaatgttgtctctgtgaggatgtaggttccatcctgggctttgctcattaggttaaggatctggcattgctgcagctcagacccagtgctgccctggttgtggcttaggccaaagctgcagctccaattcaatctctggcctgggaacctccatgtgctacaaggtgcggccttaaaaggaaaaaaaaaaaattaaatcaaggactcaagagtctttcattatttgtgttgtggaagctatatttgttttaaagtcttagttgtgtttagaaagcaagatgttcttcaactcaaatttgggagggaacttgtttcatacatttttaatggataagtggcaaaattttcatgctgaggtgatctatagtgttgtaatgcagaatatagtcagatcttgaacattttaggaagttggtgagggccaattgtgtatctgtgccatgctgataagaatgtcaagggatcacaagaattcgtgttatttgacagcagtcatctttaaaaggcatttgagaaagtccaatttcaaatgcatttcctttctttaaaagataaattgaagaaaataagtctttatttcccaagtaaattgaattgcctctcagtctgttaaaagaaactcttaccttgatgattgcgctcttaacctggcaaagattgtctttaaaatctgagctccatgtcttctgctttatttctggtgtgcctttgactccagattacagtaaatggaggactgagtatagggctaaaaagtagagagaatggatgcatattatctgtggtctccaatgtgatgaatgaagtaggcaaatactcaaaggaaagagaaagcatgctccaagaattatgggttccagaaggcaaagtcccagaattgtctccagggaaggacagggaggtctagaatcggctaagcccactgtaggcagaaaaaccaagaggcatgaatggcttccctttctcacttttcactctctggcttactcctatcatgaaggaaaatattggaatcatattctccctcaccgaaatgctatttttcagcccacaggaaacccaggctggttggaggggacattccctgctctggtcgtgttgaagtacaacatggagacacgtggggcaccgtctgtgattctgacttctctctggaggcggccagcgtgctgtgcagggaactacagtgcggcaactgtggtttccctcctggggggagctcactttggagaaggaagtggacagatctgggctgaagaattccagtgtgaggggcacgagtcccacctttcactctgcccagtagcaccccgccctgacgggacatgtagccacagcagggacgtcggcgtagtctgctcaagtgagacccagggaatgtgttcactttgttcccatgccatgaagagggtagggttaggtagtcacagacatctttttaaagccctgtctccttccaggatacacacaaatccgcttggtgaatggcaagaccccatgtgaaggaagagtggagctcaacattcttgggtcctgggggtccctctgcaactctcactgggacatggaagatgcccatgttttatgccagcagcttaaatgtggagttgccctttctatcccgggaggagcaccttttgggaaaggaagtgagcaggtctggaggcacatgtttcactgcactgggactgagaagcacatgggagattgttccgtcactgctctgggcgcatcactctgttcttcagggcaagtggcctctgtaatctgctcaggtaagagaataagggcagccagtgatgagccactcatgacggtgccttaagagtgggtgtacctaggagttcccattgtggctcagtggtaacaaactcgactggtatccatgagggtatgggtttgatccctggccttgctcaatgggttaaggatccagcattgctgtgagctgtggtataggttgcagactctgctcaggtcccatgttgctgtgattgtggtgtaggctgactgctgcagcttcaatttgacccctagcccgggaatttccataggccacacgtgcagcactaaggaaggaaaaaaagaaaaaaaaaaaaaaagagtgggtgtgcctatagtgaagaacagatgtaaaagggaagtgaaagggattcccccattctgagggattgtgagaagtgtgccagaatattaacttcatttgacttgttacagggaaagtaaacttgactttcacggacctcctagttacctggtgcttactatatgtcttctcagagtacctgattcattcccagcctggttgacccatccccctatctctatggctatgtttatccagagcacatctatctaacactccagctgatcttcctgacacagctgtggcaaccctggatcctttaaccaactgtgccaggctggagatcaaacctaagcctctgcagcaacccaagctgctgcagtcagatttttaaccccctgtgccactgtgggtatctccgatattttgtatcttctgtgactgagtggtttgctgtttgcagggaaccagagtcagacactatccccgtgcaattcatcatcctcggacccatcaagctctattatttcagaagaaaatggtgttgcctgcataggtgagaatcagtgaccaacctatgaaaatgatctcaatcctctgaaatgcattttattcatgttttatttcctctttgcagggagtggtcaacttcgcctggtcgatggaggtggtcgttgtgctgggagagtagaggtctatcatgagggctcctggggcaccatctgtgatgacagctgggacctgaatgatgcccatgtggtgtgcaaacagctgagctgtggatgggccattaatgccactggttctgctcattttggggaaggaacagggcccatttggctggatgagataaactgtaatggaaaagaatctcatatttggcaatgccactcacatggttgggggcggcacaattgcaggcataaggaggatgcaggagtcatctgctcgg

SEQ ID NO: 107 - DNA, 4860 bp, Sus scrofa
  source 1..4860: mol_type = other DNA
tatagatgacaaggctttgtgtctgataggggccagcgaactcagtaaagagggaagatgagaaagataatggcaagaatttatccctgaagtgtagttttgacaaaccagtcacaaagaggtctaagaaattttggtcacaaagttgttttgaatcccaggcattttatttgcaatgattgcatatgttctggaaaggacatctgaacctaagaaatagttcatttgcattgtgttatattttactaaggtctgagaaataatcttgagatgagaatgaactctacttcttcagagtctggaaggaataaattatgaaaatgtattaatgcttctttaaaccatattgtatatttatctattactaaacaaaaagaagtagctctatttatttatttatttatttatttatttatgtcttttgtctctttagggccacacctgtggcatatggaggttcccaggctagaggtccaattggagatgtagcagccagcctatgccagagccaccgcaacacgggatctgagccacgtctgtgacttacaccacagctcacagcaacgcctgatcctcaacccactgagcgaggccagggatcgaacccatgtcctcatggatgctagttgggttcgttaactgctgagccatgatgggaactccaaattaattatttcttatatttgttcttcatatattcatttctatagaaagaaataaatacagattcagttaatgatggcaggtaaaagcttaacttattaatcaaaggagttaatccaggcacaaaaattcaattcatggctctctgttaaaatttaggtataggtttagcaggaagaaaaggttagtagatgcagactattacatttagaatggatggacaatgaagtcctactatacagcacagggaactatatccaatctcttgggatagaatatgatggaagacaaaatcagaacaagagagtatatatatatgtgtgtgtgtgtgtgtgtgtgtgtgtgtgtgtgtgtgtgtgtgtgactgggtcaccctgcggcacagcagaaattggcagaacattgtaaatcaactatactttaataggaaaaatacttttaagggctaaatttccaatattctaaccatgtacacagagtaaatgtcataaggatgccagtctgtgtagagattgatgtgttactagcagattcatgaaataaaggctgaggatgtagtccccaagtcacttctgagtggaagaatttctcctttgtcctggactcaaatattttaggataaaggaaaaaagaagatatttatagaagggacttgttttcaagtacttgacaaaatttcaccattaaagagaaatttgtgggagttcccatcgtggctcagtggaaacaaatccaactaggaaccatgaggttgtgggtttgatccctggcctcactcagtgggttaaggatccggtgttgccgtgagctgtggtgtaggttgcagacacggttctgatcctgcgttgctgtggctgtggctgtggtgtaggccagcagcaaacagctctgattagacccctagcctggaaacctccatatgccacaggtgcagccctaaaaagacaaaaaaagagaaaagacaaaaaaaaaaaaaaaaaaaaaaaaaaaaaaaaaaaaaaaaaaaagaacccccagaggtatttatttgtttttgccttttttcactgactgttctttgtttgtttgtttgagactgatctagaagactagagattacaagaaatatggatttggctcactctaagaaactgctttcattccaaggtttgggtctatccaaaagtggaatagaatcatatgaatactagtttatgagtatttagtgagaggaatttcaagctcaaataatgattcagcaagattaaattaaggagggaattttccttgtggctgagtgggttaaggacccaatgttgtctctgtgaggatgtaggttccatcctgggctttgctcattaggttaaggatctggcattgctgcagctcagacccagtgctgccctggttgtggcttaggccaaagctgcagctccaattcaatctctggcctgggaacctccatgtgctacaaggtgcggccttaaaaggaaaaaaaaaaaattaaatcaaggactcaagagtctttcattatttgtgttgtggaagctatatttgttttaaagtcttagttgtgtttagaaagcaagatgttcttcaactcaaatttgggagggaacttgtttcatacatttttaatggataagtggcaaaattttcatgctgaggtgatctatagtgttgtaatgcagaatatagtcagatcttgaacattttaggaagttggtgagggccaattgtgtatctgtgccatgctgataagaatgtcaagggatcacaagaattcgtgttatttgacagcagtcatctttaaaaggcatttgagaaagtccaatttcaaatgcatttcctttctttaaaagataaattgaagaaaataagtctttatttcccaagtaaattgaattgcctctcagtctgttaaaagaaactcttaccttgatgattgcgctcttaacctggcaaagattgtctttaaaatctgagctccatgtcttctgctttatttctggtgtgcctttgactccagattacagtaaatggaggactgagtatagggctaaaaagtagagagaatggatgcatattatctgtggtctccaatgtgatgaatgaagtaggcaaatactcaaaggaaagagaaagcatgctccaagaattatgggttccagaaggcaaagtcccagaattgtctccagggaaggacagggaggtctagaatcggctaagcccactgtaggcagaaaaaccaagaggcatgaatggcttccctttctcacttttcactctctggcttactcctatcatgaaggaaaatattggaatcatattctccctcaccgaaatgctatttttcagcccacaggaaacccaggctggttggagggtcctggggggagctcactttggagaaggaagtggacagatctgggctgaagaattccagtgtgaggggcacgagtcccacctttcactctgcccagtagcaccccgccctgacgggacatgtagccacagcagggacgtcggcgtagtctgctcaagtgagacccagggaatgtgttcactttgttcccatgccatgaagagggtagggttaggtagtcacagacatctttttaaagccctgtctccttccaggatacacacaaatccgcttggtgaatggcaagaccccatgtgaaggaagagtggagctcaacattcttgggtcctgggggtccctctgcaactctcactgggacatggaagatgcccatgttttatgccagcagcttaaatgtggagttgccctttctatcccgggaggagcaccttttgggaaaggaagtgagcaggtctggaggcacatgtttcactgcactgggactgagaagcacatgggagattgttccgtcactgctctgggcgcatcactctgttcttcagggcaagtggcctctgtaatctgctcaggtaagagaataagggcagccagtgatgagccactcatgacggtgccttaagagtgggtgtacctaggagttcccattgtggctcagtggtaacaaactcgactggtatccatgagggtatgggtttgatccctggccttgctcaatgggttaaggatccagcattgctgtgagctgtggtataggttgcagactctgctcaggtcccatgttgctgtgattgtggtgtaggctgactgctgcagcttcaatttgacccctagcccgggaatttccataggccacacgtgcagcactaaggaaggaaaaaaagaaaaaaaaaaaaaaagagtgggtgtgcctatagtgaagaacagatgtaaaagggaagtgaaagggattcccccattctgagggattgtgagaagtgtgccagaatattaacttcatttgacttgttacagggaaagtaaacttgactttcacggacctcctagttacctggtgcttactatatgtcttctcagagtacctgattcattcccagcctggttgacccatccccctatctctatggctatgtttatccagagcacatctatctaacactccagctgatcttcctgacacagctgtggcaaccctggatcctttaaccaactgtgccaggctggagatcaaacctaagcctctgcagcaacccaagctgctgcagtcagatttttaaccccctgtgccactgtgggtatctccgatattttgtatcttctgtgactgagtggtttgctgtttgcagggaaccagagtcagacactatccccgtgcaattcatcatcctcggacccatcaagctctattatttcagaagaaaatggtgttgcctgcataggtgagaatcagtgaccaacctatgaaaatgatctcaatcctctgaaatgcattttattcatgttttatttcctctttgcagggagtggtcaacttcgcctggtcgatggaggtggtcgttgtgctgggagagtagaggtctatcatgagggctcctggggcaccatctgtgatgacagctgggacctgaatgatgcccatgtggtgtgcaaacagctgagctgtggatgggccattaatgccactggttctgctcattttggggaaggaacagggcccatttggctggatgagataaactgtaatggaaaagaatctcatatttggcaatgccactcacatggttgggggcggcacaattgcaggcataaggaggatgcaggagtcatctgctcgg

SEQ ID NO: 108 - DNA, 4858 bp, Sus scrofa
  source 1..4858: mol_type = other DNA
tatagatgacaaggctttgtgtctgataggggccagcgaactcagtaaagagggaagatgagaaagataatggcaagaatttatccctgaagtgtagttttgacaaaccagtcacaaagaggtctaagaaattttggtcacaaagttgttttgaatcccaggcattttatttgcaatgattgcatatgttctggaaaggacatctgaacctaagaaatagttcatttgcattgtgttatattttactaaggtctgagaaataatcttgagatgagaatgaactctacttcttcagagtctggaaggaataaattatgaaaatgtattaatgcttctttaaaccatattgtatatttatctattactaaacaaaaagaagtagctctatttatttatttatttatttatttatttatgtcttttgtctctttagggccacacctgtggcatatggaggttcccaggctagaggtccaattggagatgtagcagccagcctatgccagagccaccgcaacacgggatctgagccacgtctgtgacttacaccacagctcacagcaacgcctgatcctcaacccactgagcgaggccagggatcgaacccatgtcctcatggatgctagttgggttcgttaactgctgagccatgatgggaactccaaattaattatttcttatatttgttcttcatatattcatttctatagaaagaaataaatacagattcagttaatgatggcaggtaaaagcttaacttattaatcaaaggagttaatccaggcacaaaaattcaattcatggctctctgttaaaatttaggtataggtttagcaggaagaaaaggttagtagatgcagactattacatttagaatggatggacaatgaagtcctactatacagcacagggaactatatccaatctcttgggatagaatatgatggaagacaaaatcagaacaagagagtatatatatatgtgtgtgtgtgtgtgtgtgtgtgtgtgtgtgtgtgtgtgtgtgtgactgggtcaccctgcggcacagcagaaattggcagaacattgtaaatcaactatactttaataggaaaaatacttttaagggctaaatttccaatattctaaccatgtacacagagtaaatgtcataaggatgccagtctgtgtagagattgatgtgttactagcagattcatgaaataaaggctgaggatgtagtccccaagtcacttctgagtggaagaatttctcctttgtcctggactcaaatattttaggataaaggaaaaaagaagatatttatagaagggacttgttttcaagtacttgacaaaatttcaccattaaagagaaatttgtgggagttcccatcgtggctcagtggaaacaaatccaactaggaaccatgaggttgtgggtttgatccctggcctcactcagtgggttaaggatccggtgttgccgtgagctgtggtgtaggttgcagacacggttctgatcctgcgttgctgtggctgtggctgtggtgtaggccagcagcaaacagctctgattagacccctagcctggaaacctccatatgccacaggtgcagccctaaaaagacaaaaaaagagaaaagacaaaaaaaaaaaaaaaaaaaaaaaaaaaaaaaaaaaaaaaaaaaagaacccccagaggtatttatttgtttttgccttttttcactgactgttctttgtttgtttgtttgagactgatctagaagactagagattacaagaaatatggatttggctcactctaagaaactgctttcattccaaggtttgggtctatccaaaagtggaatagaatcatatgaatactagtttatgagtatttagtgagaggaatttcaagctcaaataatgattcagcaagattaaattaaggagggaattttccttgtggctgagtgggttaaggacccaatgttgtctctgtgaggatgtaggttccatcctgggctttgctcattaggttaaggatctggcattgctgcagctcagacccagtgctgccctggttgtggcttaggccaaagctgcagctccaattcaatctctggcctgggaacctccatgtgctacaaggtgcggccttaaaaggaaaaaaaaaaaattaaatcaaggactcaagagtctttcattatttgtgttgtggaagctatatttgttttaaagtcttagttgtgtttagaaagcaagatgttcttcaactcaaatttgggagggaacttgtttcatacatttttaatggataagtggcaaaattttcatgctgaggtgatctatagtgttgtaatgcagaatatagtcagatcttgaacattttaggaagttggtgagggccaattgtgtatctgtgccatgctgataagaatgtcaagggatcacaagaattcgtgttatttgacagcagtcatctttaaaaggcatttgagaaagtccaatttcaaatgcatttcctttctttaaaagataaattgaagaaaataagtctttatttcccaagtaaattgaattgcctctcagtctgttaaaagaaactcttaccttgatgattgcgctcttaacctggcaaagattgtctttaaaatctgagctccatgtcttctgctttatttctggtgtgcctttgactccagattacagtaaatggaggactgagtatagggctaaaaagtagagagaatggatgcatattatctgtggtctccaatgtgatgaatgaagtaggcaaatactcaaaggaaagagaaagcatgctccaagaattatgggttccagaaggcaaagtcccagaattgtctccagggaaggacagggaggtctagaatcggctaagcccactgtaggcagaaaaaccaagaggcatgaatggcttccctttctcacttttcactctctggcttactcctatcatgaaggaaaatattggaatcatattctccctcaccgaaatgctatttttcagcccacaggaaacccaggctggttggagggctggggggagctcactttggagaaggaagtggacagatctgggctgaagaattccagtgtgaggggcacgagtcccacctttcactctgcccagtagcaccccgccctgacgggacatgtagccacagcagggacgtcggcgtagtctgctcaagtgagacccagggaatgtgttcactttgttcccatgccatgaagagggtagggttaggtagtcacagacatctttttaaagccctgtctccttccaggatacacacaaatccgcttggtgaatggcaagaccccatgtgaaggaagagtggagctcaacattcttgggtcctgggggtccctctgcaactctcactgggacatggaagatgcccatgttttatgccagcagcttaaatgtggagttgccctttctatcccgggaggagcaccttttgggaaaggaagtgagcaggtctggaggcacatgtttcactgcactgggactgagaagcacatgggagattgttccgtcactgctctgggcgcatcactctgttcttcagggcaagtggcctctgtaatctgctcaggtaagagaataagggcagccagtgatgagccactcatgacggtgccttaagagtgggtgtacctaggagttcccattgtggctcagtggtaacaaactcgactggtatccatgagggtatgggtttgatccctggccttgctcaatgggttaaggatccagcattgctgtgagctgtggtataggttgcagactctgctcaggtcccatgttgctgtgattgtggtgtaggctgactgctgcagcttcaatttgacccctagcccgggaatttccataggccacacgtgcagcactaaggaaggaaaaaaagaaaaaaaaaaaaaaagagtgggtgtgcctatagtgaagaacagatgtaaaagggaagtgaaagggattcccccattctgagggattgtgagaagtgtgccagaatattaacttcatttgacttgttacagggaaagtaaacttgactttcacggacctcctagttacctggtgcttactatatgtcttctcagagtacctgattcattcccagcctggttgacccatccccctatctctatggctatgtttatccagagcacatctatctaacactccagctgatcttcctgacacagctgtggcaaccctggatcctttaaccaactgtgccaggctggagatcaaacctaagcctctgcagcaacccaagctgctgcagtcagatttttaaccccctgtgccactgtgggtatctccgatattttgtatcttctgtgactgagtggtttgctgtttgcagggaaccagagtcagacactatccccgtgcaattcatcatcctcggacccatcaagctctattatttcagaagaaaatggtgttgcctgcataggtgagaatcagtgaccaacctatgaaaatgatctcaatcctctgaaatgcattttattcatgttttatttcctctttgcagggagtggtcaacttcgcctggtcgatggaggtggtcgttgtgctgggagagtagaggtctatcatgagggctcctggggcaccatctgtgatgacagctgggacctgaatgatgcccatgtggtgtgcaaacagctgagctgtggatgggccattaatgccactggttctgctcattttggggaaggaacagggcccatttggctggatgagataaactgtaatggaaaagaatctcatatttggcaatgccactcacatggttgggggcggcacaattgcaggcataaggaggatgcaggagtcatctgctcgg

SEQ ID NO: 109 - DNA, 3523 bp, Sus scrofa
  source 1..3523: mol_type = other DNA
tatagatgacaaggctttgtgtctgataggggccagcgaactcagtaaagagggaagatgagaaagataatggcaagaatttatccctgaagtgtagttttgacaaaccagtcacaaagaggtctaagaaattttggtcacaaagttgttttgaatcccaggcattttatttgcaatgattgcatatgttctggaaaggacatctgaacctaagaaatagttcatttgcattgtgttatattttactaaggtctgagaaataatcttgagatgagaatgaactctacttcttcagagtctggaaggaataaattatgaaaatgtattaatgcttctttaaaccatattgtatatttatctattactaaacaaaaagaagtagctctatttatttatttatttatttatttatttatgtcttttgtctctttagggccacacctgtggcatatggaggttcccaggctagaggtccaattggagatgtagcagccagcctatgccagagccaccgcaacacgggatctgagccacgtctgtgacttacaccacagctcacagcaacgcctgatcctcaacccactgagcgaggccagggatcgaacccatgtcctcatggatgctagttgggttcgttaactgctgagccatgatgggaactccaaattaattatttcttatatttgttcttcatatattcatttctatagaaagaaataaatacagattcagttaatgatggcaggtaaaagcttaacttattaatcaaaggagttaatccaggcacaaaaattcaattcatggctctctgttaaaatttaggtataggtttagcaggaagaaaaggttagtagatgcagactattacatttagaatggatggacaatgaagtcctactatacagcacagggaactatatccaatctcttgggatagaatatgatggaagacaaaatcagaacaagagagtatatatatatgtgtgtgtgtgtgtgtgtgtgtgtgtgtgtgtgtgtgtgtgtgtgactgggtcaccctgcggcacagcagaaattggcagaacattgtaaatcaactatactttaataggaaaaatacttttaagggctaaatttccaatattctaaccatgtacacagagtaaatgtcataaggatgccagtctgtgtagagattgatgtgttactagcagattcatgaaataaaggctgaggatgtagtccccaagtcacttctgagtggaagaatttctcctttgtcctggactcaaatattttaggataaaggaaaaaagaagatatttatagaagggacttgttttcaagtacttgacaaaatttcaccattaaagagaaatttgtgggagttcccatcgtggctcagtggaaacaaatccaactaggaaccatgaggttgtgggtttgatccctggcctcactcagtgggttaaggatccggtgttgccgtgagctgtggtgtaggttgcagacacggttctgatcctgcgttgctgtggctgtggctgtggtgtaggccagcagcaaacagctctgattagacccctagcctggaaacctccatatgccacaggtgcagccctaaaaagacaaaaaaagagaaaagacaaaaaaaaaaaaaaaaaaaaaaaaaaaaaaaaaaaaaaaaaaaagaacccccagaggtatttatttgtttttgccttttttcactgactgttctttgtttgtttgtttgagactgatctagaagactagagattacaagaaatatggatttggctcactctaagaaactgctttcattccaaggtttgggtctatccaaaagtggaatagaatcatatgaatactagtttatgagtatttagtgagaggaatttcaagctcaaataatgattcagcaagattaaattaaggagggaattttccttgtggctgagtgggttaaggacccaatgttgtctctgtgaggatgtaggttccatcctgggctttgctcattaggttaaggatctggcattgctgcagctcagacccagtgctgccctggttgtggcttaggccaaagctgcagctccaattcaatctctggcctgggaacctccatgtgctacaaggtgcggccttaaaaggaaaaaaaaaaaattaaatcaaggactcaagagtctttcattatttgtgttgtggaagctatatttgttttaaagtcttagttgtgtttagaaagcaagatgttcttcaactcaaatttgggagggaacttgtttcatacatttttaatggataagtggcaaaattttcatgctgaggtgatctatagtgttgtaatgcagaatatagtcagatcttgaacattttaggaagttggtgagggccaattgtgtatctgtgccatgctgataagaatgtcaagggatcacaagaattcgtgagctgtggtataggttgcagactctgctcaggtcccatgttgctgtgattgtggtgtaggctgactgctgcagcttcaatttgacccctagcccgggaatttccataggccacacgtgcagcactaaggaaggaaaaaaagaaaaaaaaaaaaaaagagtgggtgtgcctatagtgaagaacagatgtaaaagggaagtgaaagggattcccccattctgagggattgtgagaagtgtgccagaatattaacttcatttgacttgttacagggaaagtaaacttgactttcacggacctcctagttacctggtgcttactatatgtcttctcagagtacctgattcattcccagcctggttgacccatccccctatctctatggctatgtttatccagagcacatctatctaacactccagctgatcttcctgacacagctgtggcaaccctggatcctttaaccaactgtgccaggctggagatcaaacctaagcctctgcagcaacccaagctgctgcagtcagatttttaaccccctgtgccactgtgggtatctccgatattttgtatcttctgtgactgagtggtttgctgtttgcagggaaccagagtcagacactatccccgtgcaattcatcatcctcggacccatcaagctctattatttcagaagaaaatggtgttgcctgcataggtgagaatcagtgaccaacctatgaaaatgatctcaatcctctgaaatgcattttattcatgttttatttcctctttgcagggagtggtcaacttcgcctggtcgatggaggtggtcgttgtgctgggagagtagaggtctatcatgagggctcctggggcaccatctgtgatgacagctgggacctgaatgatgcccatgtggtgtgcaaacagctgagctgtggatgggccattaatgccactggttctgctcattttggggaaggaacagggcccatttggctggatgagataaactgtaatggaaaagaatctcatatttggcaatgccactcacatggttgggggcggcacaattgcaggcataaggaggatgcaggagtcatctgctcgg

SEQ ID NO: 110 - DNA, 3603 bp, Sus scrofa
  source 1..3603: mol_type = other DNA
tatagatgacaaggctttgtgtctgataggggccagcgaactcagtaaagagggaagatgagaaagataatggcaagaatttatccctgaagtgtagttttgacaaaccagtcacaaagaggtctaagaaattttggtcacaaagttgttttgaatcccaggcattttatttgcaatgattgcatatgttctggaaaggacatctgaacctaagaaatagttcatttgcattgtgttatattttactaaggtctgagaaataatcttgagatgagaatgaactctacttcttcagagtctggaaggaataaattatgaaaatgtattaatgcttctttaaaccatattgtatatttatctattactaaacaaaaagaagtagctctatttatttatttatttatttatttatttatgtcttttgtctctttagggccacacctgtggcatatggaggttcccaggctagaggtccaattggagatgttgtggagaattccacaagaattcgtgttatttgacagcagtcatctttaaaaggcatttgagaaagtccaatttcaaatgcatttcctttctttaaaagataaattgaagaaaataagtctttatttcccaagtaaattgaattgcctctcagtctgttaaaagaaactcttatatagatgacaaggctttgtgtctgataggggccagcgaactcagtaaagagggaagatgagaaagataatggcaagaatttatccctgaagtgtagttttgacaaaccagtcacaaagaggtctaagaaattttggtcacaaagttgttttgaatcccaggcattttatttgcaatgattgcatatgttctggaaaggacatctgaacctaagaaatagttcatttgcattgtgttatattttactaaggtctgagaaataatcttgagatgagaatgaactctacttcttcagagtctggaaggaataaattatgaaaatgtattaatgcttctttaaaccatattgtatatttatctattactaaacaaaaagaagtagctctatttatttatttatttatttatttatttatgtcttttgtctctttagggccacacctgtggcatatggaggttcccaggctagaggtccaattggagatgttgtggagaattccacaagaattcgtgttatttgacagcagtcatctttaaaaggcatttgagaaagtccaatttcaaatgcatttcctttctttaaaagataaattgaagaaaataagtctttatttcccaagtaaattgaattgcctctcagtctgttaaaagaaactcttaccttgatgattgcgctcttaacctggcaaagattgtctttaaaatctgagctccatgtcttctgctttatttctggtgtgcctttgactccagattacagtaaatggaggactgagtatagggctaaaaagtagagagaatggatgcatattatctgtggtctccaatgtgatgaatgaagtaggcaaatactcaaaggaaagagaaagcatgctccaagaattatgggttccagaaggcaaagtcccagaattgtctccagggaaggacagggaggtctagaatcggctaagcccactgtaggcagaaaaaccaagaggcatgaatggcttccctttctcacttttcactctctggcttactcctatcatgaaggaaaatattggaatcatattctccctcaccgaaatgctatttttcagcccacaggaaacccaggctggttggaggggacattccctgctctcactttggagaaggaagtggacagatctgggctgaagaattccagtgtgaggggcacgagtcccacctttcactctgcccagtagcaccccgccctgacgggacatgtagccacagcagggacgtcggcgtagtctgctcaagtgagacccagggaatgtgttcactttgttcccatgccatgaagagggtagggttaggtagtcacagacatctttttaaagccctgtctccttccaggatacacacaaatccgcttggtgaatggcaagaccccatgtgaaggaagagtggagctcaacattcttgggtcctgggggtccctctgcaactctcactgggacatggaagatgcccatgttttatgccagcagcttaaatgtggagttgccctttctatcccgggaggagcaccttttgggaaaggaagtgagcaggtctggaggcacatgtttcactgcactgggactgagaagcacatgggagattgttccgtcactgctctgggcgcatcactctgttcttcagggcaagtggcctctgtaatctgctcaggtaagagaataagggcagccagtgatgagccactcatgacggtgccttaagagtgggtgtacctaggagttcccattgtggctcagtggtaacaaactcgactggtatccatgagggtatgggtttgatccctggccttgctcaatgggttaaggatccagcattgctgtgagctgtggtataggttgcagactctgctcaggtcccatgttgctgtgattgtggtgtaggctgactgctgcagcttcaatttgacccctagcccgggaatttccataggccacacgtgcagcactaaggaaggaaaaaaagaaaaaaaaaaaaaaagagtgggtgtgcctatagtgaagaacagatgtaaaagggaagtgaaagggattcccccattctgagggattgtgagaagtgtgccagaatattaacttcatttgacttgttacagggaaagtaaacttgactttcacggacctcctagttacctggtgcttactatatgtcttctcagagtacctgattcattcccagcctggttgacccatccccctatctctatggctatgtttatccagagcacatctatctaacactccagctgatcttcctgacacagctgtggcaaccctggatcctttaaccaactgtgccaggctggagatcaaacctaagcctctgcagcaacccaagctgctgcagtcagatttttaaccccctgtgccactgtgggtatctccgatattttgtatcttctgtgactgagtggtttgctgtttgcagggaaccagagtcagacactatccccgtgcaattcatcatcctcggacccatcaagctctattatttcagaagaaaatggtgttgcctgcataggtgagaatcagtgaccaacctatgaaaatgatctcaatcctctgaaatgcattttattcatgttttatttcctctttgcagggagtggtcaacttcgcctggtcgatggaggtggtcgttgtgctgggagagtagaggtctatcatgagggctcctggggcaccatctgtgatgacagctgggacctgaatgatgcccatgtggtgtgcaaacagctgagctgtggatgggccattaatgccactggttctgctcattttggggaaggaacagggcccatttggctggatgagataaactgtaatggaaaagaatctcatatttggcaatgccactcacatggttgggggcggcacaattgcaggcataaggaggatgcaggagtcatctgctcgg

SEQ ID NO: 111 - DNA, 4962 bp, Sus scrofa
  source 1..4962: mol_type = other DNA
tatagatgacaaggctttgtgtctgataggggccagcgaactcagtaaagagggaagatgagaaagataatggcaagaatttatccctgaagtgtagttttgacaaaccagtcacaaagaggtctaagaaattttggtcacaaagttgttttgaatcccaggcattttatttgcaatgattgcatatgttctggaaaggacatctgaacctaagaaatagttcatttgcattgtgttatattttactaaggtctgagaaataatcttgagatgagaatgaactctacttcttcagagtctggaaggaataaattatgaaaatgtattaatgcttctttaaaccatattgtatatttatctattactaaacaaaaagaagtagctctatttatttatttatttatttatttatttatgtcttttgtctctttagggccacacctgtggcatatggaggttcccaggctagaggtccaattggagatgtagcagccagcctatgccagagccaccgcaacacgggatctgagccacgtctgtgacttacaccacagctcacagcaacgcctgatcctcaacccactgagcgaggccagggatcgaacccatgtcctcatggatgctagttgggttcgttaactgctgagccatgatgggaactccaaattaattatttcttatatttgttcttcatatattcatttctatagaaagaaataaatacagattcagttaatgatggcaggtaaaagcttaacttattaatcaaaggagttaatccaggcacaaaaattcaattcatggctctctgttaaaatttaggtataggtttagcaggaagaaaaggttagtagatgcagactattacatttagaatggatggacaatgaagtcctactatacagcacagggaactatatccaatctcttgggatagaatatgatggaagacaaaatcagaacaagagagtatatatatatgtgtgtgtgtgtgtgtgtgtgtgtgtgtgtgtgtgtgtgtgtgtgactgggtcaccctgcggcacagcagaaattggcagaacattgtaaatcaactatactttaataggaaaaatacttttaagggctaaatttccaatattctaaccatgtacacagagtaaatgtcataaggatgccagtctgtgtagagattgatgtgttactagcagattcatgaaataaaggctgaggatgtagtccccaagtcacttctgagtggaagaatttctcctttgtcctggactcaaatattttaggataaaggaaaaaagaagatatttatagaagggacttgttttcaagtacttgacaaaatttcaccattaaagagaaatttgtgggagttcccatcgtggctcagtggaaacaaatccaactaggaaccatgaggttgtgggtttgatccctggcctcactcagtgggttaaggatccggtgttgccgtgagctgtggtgtaggttgcagacacggttctgatcctgcgttgctgtggctgtggctgtggtgtaggccagcagcaaacagctctgattagacccctagcctggaaacctccatatgccacaggtgcagccctaaaaagacaaaaaaagagaaaagacaaaaaaaaaaaaaaaaaaaaaaaaaaaaaaaaaaaaaaaaaaaagaacccccagaggtatttatttgtttttgccttttttcactgactgttctttgtttgtttgtttgagactgatctagaagactagagattacaagaaatatggatttggctcactctaagaaactgctttcattccaaggtttgggtctatccaaaagtggaatagaatcatatgaatactagtttatgagtatttagtgagaggaatttcaagctcaaataatgattcagcaagattaaattaaggagggaattttccttgtggctgagtgggttaaggacccaatgttgtctctgtgaggatgtaggttccatcctgggctttgctcattaggttaaggatctggcattgctgcagctcagacccagtgctgccctggttgtggcttaggccaaagctgcagctccaattcaatctctggcctgggaacctccatgtgctacaaggtgcggccttaaaaggaaaaaaaaaaaattaaatcaaggactcaagagtctttcattatttgtgttgtggaagctatatttgttttaaagtcttagttgtgtttagaaagcaagatgttcttcaactcaaatttgggagggaacttgtttcatacatttttaatggataagtggcaaaattttcatgctgaggtgatctatagtgttgtaatgcagaatatagtcagatcttgaacattttaggaagttggtgagggccaattgtgtatctgtgccatgctgataagaatgtcaagggatcacaagaattcgtgttatttgacagcagtcatctttaaaaggcatttgagaaagtccaatttcaaatgcatttcctttctttaaaagataaattgaagaaaataagtctttatttcccaagtaaattgaattgcctctcagtctgttaaaagaaactcttaccttgatgattgcgctcttaacctggcaaagattgtctttaaaatctgagctccatgtcttctgctttatttctggtgtgcctttgactccagattacagtaaatggaggactgagtatagggctaaaaagtagagagaatggatgcatattatctgtggtctccaatgtgatgaatgaagtaggcaaatactcaaaggaaagagaaagcatgctccaagaattatgggttccagaaggcaaagtcccagaattgtctccagggaaggacagggaggtctagaatcggctaagcccactgtaggcagaaaaaccaagaggcatgaatggcttccctttctcacttttcactctctggcttactcctatcatgaaggaaaatattggaatcatattctccctcaccgaaatgctatttttcagcccacaggaaacccaggctggttggaggggacattccctgctctggtcgtgttgaagtacaacatggagacacgtggggcaccgtctgtgattctgacttctctctggaggcggccagcgtgctgtgcagggaactacagtgcgtcactttggagaaggaagtggacagatctgggctgaagaattccagtgtgaggggcacgagtcccacctttcactctgcccagtagcaccccgccctgacgggacatgtagccacagcagggacgtcggcgtagtctgctcaagtgagacccagggaatgtgttcactttgttcccatgccatgaagagggtagggttaggtagtcacagacatctttttaaagccctgtctccttccaggatacacacaaatccgcttggtgaatggcaagaccccatgtgaaggaagagtggagctcaacattcttgggtcctgggggtccctctgcaactctcactgggacatggaagatgcccatgttttatgccagcagcttaaatgtggagttgccctttctatcccgggaggagcaccttttgggaaaggaagtgagcaggtctggaggcacatgtttcactgcactgggactgagaagcacatgggagattgttccgtcactgctctgggcgcatcactctgttcttcagggcaagtggcctctgtaatctgctcaggtaagagaataagggcagccagtgatgagccactcatgacggtgccttaagagtgggtgtacctaggagttcccattgtggctcagtggtaacaaactcgactggtatccatgagggtatgggtttgatccctggccttgctcaatgggttaaggatccagcattgctgtgagctgtggtataggttgcagactctgctcaggtcccatgttgctgtgattgtggtgtaggctgactgctgcagcttcaatttgacccctagcccgggaatttccataggccacacgtgcagcactaaggaaggaaaaaaagaaaaaaaaaaaaaaagagtgggtgtgcctatagtgaagaacagatgtaaaagggaagtgaaagggattcccccattctgagggattgtgagaagtgtgccagaatattaacttcatttgacttgttacagggaaagtaaacttgactttcacggacctcctagttacctggtgcttactatatgtcttctcagagtacctgattcattcccagcctggttgacccatccccctatctctatggctatgtttatccagagcacatctatctaacactccagctgatcttcctgacacagctgtggcaaccctggatcctttaaccaactgtgccaggctggagatcaaacctaagcctctgcagcaacccaagctgctgcagtcagatttttaaccccctgtgccactgtgggtatctccgatattttgtatcttctgtgactgagtggtttgctgtttgcagggaaccagagtcagacactatccccgtgcaattcatcatcctcggacccatcaagctctattatttcagaagaaaatggtgttgcctgcataggtgagaatcagtgaccaacctatgaaaatgatctcaatcctctgaaatgcattttattcatgttttatttcctctttgcagggagtggtcaacttcgcctggtcgatggaggtggtcgttgtgctgggagagtagaggtctatcatgagggctcctggggcaccatctgtgatgacagctgggacctgaatgatgcccatgtggtgtgcaaacagctgagctgtggatgggccattaatgccactggttctgctcattttggggaaggaacagggcccatttggctggatgagataaactgtaatggaaaagaatctcatatttggcaatgccactcacatggttgggggcggcacaattgcaggcataaggaggatgcaggagtcatctgctcgg

SEQ ID NO: 112 - DNA, 3603 bp, Sus scrofa
  source 1..3603: mol_type = other DNA
tatagatgacaaggctttgtgtctgataggggccagcgaactcagtaaagagggaagatgagaaagataatggcaagaatttatccctgaagtgtagttttgacaaaccagtcacaaagaggtctaagaaattttggtcacaaagttgttttgaatcccaggcattttatttgcaatgattgcatatgttctggaaaggacatctgaacctaagaaatagttcatttgcattgtgttatattttactaaggtctgagaaataatcttgagatgagaatgaactctacttcttcagagtctggaaggaataaattatgaaaatgtattaatgcttctttaaaccatattgtatatttatctattactaaacaaaaagaagtagctctatttatttatttatttatttatttatttatgtcttttgtctctttagggccacacctgtggcatatggaggttcccaggctagaggtccaattggagatgtagcagccagcctatgccagagccaccgcaacacgggatctgagccacgtctgtgacttacaccacagctcacagcaacgcctgatcctcaacccactgagcgaggccagggatcgaacccatgtcctcatggatgctagttgggttcgttaactgctgagccatgatgggaactccaaattaattatttcttatatttgttcttcatatattcatttctatagaaagaaataaatacagattcagttaatgatggcaggtaaaagcttaacttattaatcaaaggagttaatccaggcacaaaaattcaattcatggctctctgttaaaatttaggtataggtttagcaggaagaaaaggttagtagatgcagactattacatttagaatggatggacaatgaagtcctactatacagcacagggaactatatccaatctcttgggatagaatatgatggaagacaaaatcagaacaagagagtatatatatatgtgtgtgtgtgtgtgtgtgtgtgtgtgtgtgtgtgtgtgtgtgtgactgggtcaccctgcggcacagcagaaattggcagaacattgtaaatcaactatactttaataggaaaaatacttttaagggctaaatttccaatattctaaccatgtacacagagtaaatgtcataaggatgccagtctgtgtagagattgatgtgttactagcagattcatgaaataaaggctgaggatgtagtccccaagtcacttctgagtggaagaatttctcctttgtcctggactcaaatattttaggataaaggaaaaaagaagatatttatagaagggacttgttttcaagtacttgacaaaatttcaccattaaagagaaatttgtgggagttcccatcgtggctcagtggaaacaaatccaactaggaaccatgaggttgtgggtttgatccctggcctcactcagtgggttaaggatccggtgttgccgtgagctgtggtgtaggttgcagacacggttctgatcctgcgttgctgtggctgtggctgtggtgtaggccagcagcaaacagctctgattagacccctagcctggaaacctccatatgccacaggtgcagccctaaaaagacaaaaaaagagaaaagacaaaaaaaaaaaaaaaaaaaaaaaaaaaaaaaaaaaaaaaaaaaagaacccccagaggtatttatttgtttttgccttttttcactgactgttctttgtttgtttgtttgagactgatctagaagactagagattacaagaaatatggatttggctcactctaagaaactgctttcattccaaggtttgggtctatccaaaagtggaatagaatcatatgaatactagtttatgagtatttagtgagaggaatttcaagctcaaataatgattcagcaagattaaattaaggagggaattttccttgtggctgagtgggttaaggacccaatgttgtctctgtgaggatgtaggttccatcctgggctttgctcattaggttaaggatctggcattgctgcagctcagacccagtgctgccctggttgtggcttaggccaaagctgcagctccaattcaatctctggcctgggaacctccatgtgctacaaggtgcggccttaaaaggaaaaaaaaaaaattaaatcaaggactcaagagtctttcattatttgtgttgtggaagctatatttgttttaaagtcttagttgtgtttagaaagcaagatgttcttcaactcaaatttgggagggaacttgtttcatacatttttaatggataagtggcaaaattttcatgctgaggtgatctatagtgttgtaatgcagaatatagtcagatcttgaacattttaggaagttggtgagggccaattgtgtatctgtgccatgctgataagaatgtcaagggatcacaagaattcgtgttatttgacagcagtcatctttaaaaggcatttgagaaagtccaatttcaaatgcatttcctttctttaaaagataaattgaagaaaataagtctttatttcccaagtaaattgaattgcctctcagtctgttaaaagaaactcttaccttgatgattgcgctcttaacctggcaaagattgtctttaaaatctgagctccatgtcttctgctttatttctggtgtgcctttgactccagattacagtaaatggaggactgagtatagggctaaaaagtagagagaatggatgcatattatctgtggtctccaatgtgatgaatgaagtaggcaaatactcaaaggaaagagaaagcatgctccaagaattatgggttccagaaggcaaagtcccagaattgtctccagggaaggacagggaggtctagaatcggctaagcccactgtaggcagaaaaaccaagaggcatgaatggcttccctttctcacttttcactctctggcttactcctatcatgaaggaaaatattggaatcatattctccctcaccgaaatgctatttttcagcccacaggaaacccaggctggttggaggggacattccctgctctggtcgtgttgaagtacaacatggagacacgtggggcaccgtctgtgattctgacttctctctggaggcggccagcgtgctgtgcagggaactacagtgcgattcatcatcctcggacccatcaagctctattatttcagaagaaaatggtgttgcctgcataggtgagaatcagtgaccaacctatgaaaatgatctcaatcctctgaaatgcattttattcatgttttatttcctctttgcagggagtggtcaacttcgcctggtcgatggaggtggtcgttgtgctgggagagtagaggtctatcatgagggctcctggggcaccatctgtgatgacagctgggacctgaatgatgcccatgtggtgtgcaaacagctgagctgtggatgggccattaatgccactggttctgctcattttggggaaggaacagggcccatttggctggatgagataaactgtaatggaaaagaatctcatatttggcaatgccactcacatggttgggggcggcacaattgcaggcataaggaggatgcaggagtcatctgctcgg

SEQ ID NO: 113 - DNA, 3619 bp, Sus scrofa
  source 1..3619: mol_type = other DNA
tatagatgacaaggctttgtgtctgataggggccagcgaactcagtaaagagggaagatgagaaagataatggcaagaatttatccctgaagtgtagttttgacaaaccagtcacaaagaggtctaagaaattttggtcacaaagttgttttgaatcccaggcattttatttgcaatgattgcatatgttctggaaaggacatctgaacctaagaaatagttcatttgcattgtgttatattttactaaggtctgagaaataatcttgagatgagaatgaactctacttcttcagagtctggaaggaataaattatgaaaatgtattaatgcttctttaaaccatattgtatatttatctattactaaacaaaaagaagtagctctatttatttatttatttatttatttatttatgtcttttgtctctttagggccacacctgtggcatatggaggttcccaggctagaggtccaattggagatgtagcagccagcctatgccagagccaccgcaacacgggatctgagccacgtctgtgacttacaccacagctcacagcaacgcctgatcctcaacccactgagcgaggccagggatcgaacccatgtcctcatggatgctagttgggttcgttaactgctgagccatgatgggaactccaaattaattatttcttatatttgttcttcatatattcatttctatagaaagaaataaatacagattcagttaatgatggcaggtaaaagcttaacttattaatcaaaggagttaatccaggcacaaaaattcaattcatggctctctgttaaaatttaggtataggtttagcaggaagaaaaggttagtagatgcagactattacatttagaatggatggacaatgaagtcctactatacagcacagggaactatatccaatctcttgggatagaatatgatggaagacaaaatcagaacaagagagtatatatatatgtgtgtgtgtgtgtgtgtgtgtgtgtgtgtgtgtgtgtgtgtgtgactgggtcaccctgcggcacagcagaaattggcagaacattgtaaatcaactatactttaataggaaaaatacttttaagggctaaatttccaatattctaaccatgtacacagagtaaatgtcataaggatgccagtctgtgtagagattgatgtgttactagcagattcatgaaataaaggctgaggatgtagtccccaagtcacttctgagtggaagaatttctcctttgtcctggactcaaatattttaggataaaggaaaaaagaagatatttatagaagggacttgttttcaagtacttgacaaaatttcaccattaaagagaaatttgtgggagttcccatcgtggctcagtggaaacaaatccaactaggaaccatgaggttgtgggtttgatccctggcctcactcagtgggttaaggatccggtgttgccgtgagctgtggtgtaggttgcagacacggttctgatcctgcgttgctgtggctgtggctgtggtgtaggccagcagcaaacagctctgattagacccctagcctggaaacctccatatgccacaggtgcagccctaaaaagacaaaaaaagagaaaagacaaaaaaaaaaaaaaaaaaaaaaaaaaaaaaaaaaaaaaaaaaaagaacccccagaggtatttatttgtttttgccttttttcactgactgttctttgtttgtttgtttgagactgatctagaagactagagattacaagaaatatggatttggctcactctaagaaactgctttcattccaaggtttgggtctatccaaaagtggaatagaatcatatgaatactagtttatgagtatttagtgagaggaatttcaagctcaaataatgattcagcaagattaaattaaggagggaattttccttgtggctgagtgggttaaggacccaatgttgtctctgtgaggatgtaggttccatcctgggctttgctcattaggttaaggatctggcattgctgcagctcagacccagtgctgccctggttgtggcttaggccaaagctgcagctccaattcaatctctggcctgggaacctccatgtgctacaaggtgcggccttaaaaggaaaaaaaaaaaattaaatcaaggactcaagagtctttcattatttgtgttgtggaagctatatttgttttaaagtcttagttgtgtttagaaagcaagatgttcttcaactcaaatttgggagggaacttgtttcatacatttttaatggataagtggcaaaattttcatgctgaggtgatctatagtgttgtaatgcagaatatagtcagatcttgaacattttaggaagttggtgagggccaattgtgtatctgtgccatgctgataagaatgtcaagggatcacaagaattcgtgttatttgacagcagtcatctttaaaaggcatttgagaaagtccaatttcaaatgcatttcctttctttaaaagataaattgaagaaaataagtctttatttcccaagtaaattgaattgcctctcagtctgttaaaagaaactcttaccttgatgattgcgctcttaacctggcaaagattgtctttaaaatctgagctccatgtcttctgctttatttctggtgtgcctttgactccagattacagtaaatggaggactgagtatagggctaaaaagtagagagaatggatgcatattatctgtggtctccaatgtgatgaatgaagtaggcaaatactcaaaggaaagagaaagcatgctccaagaattatgggttccagaaggcaaagtcccagaattgtctccagggaaggacagggaggtctagaatcggctaagcccactgtaggcagaaaaaccaagaggcatgaatggcttccctttctcacttttcactctctggcttactcctatcatgaaggaaaatattggaatcatattctccctcaccgaaatgctatttttcagcccacaggaaacccaggctggttggaggggacattccctgctctggtcgtgttgaagtacaacatggagacacgtggggcaccgtctgtgattctgacttctctctggaggcagccagcgtgctttgcagggaaccagagtcagacactatccccgtgcaattcatcatcctcggacccatcaagctctattatttcagaagaaaatggtgttgcctgcataggtgagaatcagtgaccaacctatgaaaatgatctcaatcctctgaaatgcattttattcatgttttatttcctctttgcagggagtggtcaacttcgcctggtcgatggaggtggtcgttgtgctgggagagtagaggtctatcatgagggctcctggggcaccatctgtgatgacagctgggacctgaatgatgcccatgtggtgtgcaaacagctgagctgtggatgggccattaatgccactggttctgctcattttggggaaggaacagggcccatttggctggatgagataaactgtaatggaaaagaatctcatatttggcaatgccactcacatggttgggggcggcacaattgcaggcataaggaggatgcaggagtcatctgctcgg

SEQ ID NO: 114 - DNA, 3270 bp, Sus scrofa
  source 1..3270: mol_type = other DNA
tatagatgacaaggctttgtgtctgataggggccagcgaactcagtaaagagggaagatgagaaagataatggcaagaatttatccctgaagtgtagttttgacaaaccagtcacaaagaggtctaagaaattttggtcacaaagttgttttgaatcccaggcattttatttgcaatgattgcatatgttctggaaaggacatctgaacctaagaaatagttcatttgcattgtgttatattttactaaggtctgagaaataatcttgagatgagaatgaactctacttcttcagagtctggaaggaataaattatgaaaatgtattaatgcttctttaaaccatattgtatatttatctattactaaacaaaaagaagtagctctatttatttatttatttatttatttatttatgtcttttgtctctttagggccacacctgtggcatatggaggttcccaggctagaggtccaattggagatgtagcagccagcctatgccagagccaccgcaacacgggatctgagccacgtctgtgacttacaccacagctcacagcaacgcctgatcctcaacccactgagcgaggccagggatcgaacccatgtcctcatggatgctagttgggttcgttaactgctgagccatgatgggaactccaaattaattatttcttatatttgttcttcatatattcatttctatagaaagaaataaatacagattcagttaatgatggcaggtaaaagcttaacttattaatcaaaggagttaatccaggcacaaaaattcaattcatggctctctgttaaaatttaggtataggtttagcaggaagaaaaggttagtagatgcagactattacatttagaatggatggacaatgaagtcctactatacagcacagggaactatatccaatctcttgggatagaatatgatggaagacaaaatcagaacaagagagtatatatatatgtgtgtgtgtgtgtgtgtgtgtgtgtgtgtgtgtgtgtgtgtgtgactgggtcaccctgcggcacagcagaaattggcagaacattgtaaatcaactatactttaataggaaaaatacttttaagggctaaatttccaatattctaaccatgtacacagagtaaatgtcataaggatgccagtctgtgtagagattgatgtgttactagcagattcatgaaataaaggctgaggatgtagtccccaagtcacttctgagtggaagaatttctcctttgtcctggactcaaatattttaggataaaggaaaaaagaagatatttatagaagggacttgttttcaagtacttgacaaaatttcaccattaaagagaaatttgtgggagttcccatcgtggctcagtggaaacaaatccaactaggaaccatgaggttgtgggtttgatccctggcctcactcagtgggttaaggatccggtgttgccgtgagctgtggtgtaggttgcagacacggttctgatcctgcgttgctgtggctgtggctgtggtgtaggccagcagcaaacagctctgattagacccctagcctggaaacctccatatgccacaggtgcagccctaaaaagacaaaaaaagagaaaagacaaaaaaaaaaaaaaaaaaaaaaaaaaaaaaaaaaaaaaaaaaaagaacccccagaggtatttatttgtttttgccttttttcactgactgttctttgtttgtttgtttgagactgatctagaagactagagattacaagaaatatggatttggctcactctaagaaactgctttcattccaaggtttgggtctatccaaaagtggaatagaatcatatgaatactagtttatgagtatttagtgagaggaatttcaagctcaaataatgattcagcaagattaaattaaggagggaattttccttgtggctgagtgggttaaggacccaatgttgtctctgtgaggatgtaggttccatcctgggctttgctcattaggttaaggatctggcattgctgcagctcagacccagtgctgccctggttgtggcttaggccaaagctgcagctccaattcaatctctggcctgggaacctccatgtgctacaaggtgcggccttaaaaggaaaaaaaaaaaattaaatcaaggactcaagagtctttcattatttgtgttgtggaagctatatttgttttaaagtcttagttgtgtttagaaagcaagatgttcttcaactcaaatttgggagggaacttgtttcatacatttttaatggataagtggcaaaattttcatgctgaggtgatctatagtgttgtaatgcagaatatagtcagatcttgaacattttaggaagttggtgagggccaattgtgtatctgtgccatgctgataagaatgtcaagggatcacaagaattcgtgttatttgacttgttacagggaaagtaaacttgactttcacggacctcctagttacctggtgcttactatatgtcttctcagagtacctgattcattcccagcctggttgacccatccccctatctctatggctatgtttatccagagcacatctatctaacactccagctgatcttcctgacacagctgtggcaaccctggatcctttaaccaactgtgccaggctggagatcaaacctaagcctctgcagcaacccaagctgctgcagtcagatttttaaccccctgtgccactgtgggtatctccgatattttgtatcttctgtgactgagtggtttgctgtttgcagggaaccagagtcagacactatccccgtgcaattcatcatcctcggacccatcaagctctattatttcagaagaaaatggtgttgcctgcataggtgagaatcagtgaccaacctatgaaaatgatctcaatcctctgaaatgcattttattcatgttttatttcctctttgcagggagtggtcaacttcgcctggtcgatggaggtggtcgttgtgctgggagagtagaggtctatcatgagggctcctggggcaccatctgtgatgacagctgggacctgaatgatgcccatgtggtgtgcaaacagctgagctgtggatgggccattaatgccactggttctgctcattttggggaaggaacagggcccatttggctggatgagataaactgtaatggaaaagaatctcatatttggcaatgccactcacatggttgggggcggcacaattgcaggcataaggaggatgcaggagtcatctgctcgg

SEQ ID NO: 115 - skipped

SEQ ID NO: 116 - DNA, 12 bp, Sus scrofa
  source 1..12: mol_type = other DNA
tgtggagaattc

SEQ ID NO: 117 - DNA, 11 bp, Sus scrofa
  source 1..11: mol_type = other DNA
agccagcgtgc

SEQ ID NO: 118 - DNA, 8532 bp, Sus scrofa
  source 1..8532: mol_type = other DNA
tatagatgacaaggctttgtgtctgataggggccagcgaactcagtaaagagggaagatgagaaagataatggcaagaatttatccctgaagtgtagttttgacaaaccagtcacaaagaggtctaagaaattttggtcacaaagttgttttgaatcccaggcattttatttgcaatgattgcatatgttctggaaaggacatctgaacctaagaaatagttcatttgcattgtgttatattttactaaggtctgagaaataatcttgagatgagaatgaactctacttcttcagagtctggaaggaataaattatgaaaatgtattaatgcttctttaaaccatattgtatatttatctattactaaacaaaaagaagtagctctatttatttatttatttatttatttatttatgtcttttgtctctttagggccacacctgtggcatatggaggttcccaggctagaggtccaattggagatgtagcagccagcctatgccagagccaccgcaacacgggatctgagccacgtctgtgacttacaccacagctcacagcaacgcctgatcctcaacccactgagcgaggccagggatcgaacccatgtcctcatggatgctagttgggttcgttaactgctgagccatgatgggaactccaaattaattatttcttatatttgttcttcatatattcatttctatagaaagaaataaatacagattcagttaatgatggcaggtaaaagcttaacttattaatcaaaggagttaatccaggcacaaaaattcaattcatggctctctgttaaaatttaggtataggtttagcaggaagaaaaggttagtagatgcagactattacatttagaatggatggacaatgaagtcctactatacagcacagggaactatatccaatctcttgggatagaatatgatggaagacaaaatcagaacaagagagtatatatatatgtgtgtgtgtgtgtgtgtgtgtgtgtgtgtgtgtgtgtgtgtgtgactgggtcaccctgcggcacagcagaaattggcagaacattgtaaatcaactatactttaataggaaaaatacttttaagggctaaatttccaatattctaaccatgtacacagagtaaatgtcataaggatgccagtctgtgtagagattgatgtgttactagcagattcatgaaataaaggctgaggatgtagtccccaagtcacttctgagtggaagaatttctcctttgtcctggactcaaatattttaggataaaggaaaaaagaagatatttatagaagggacttgttttcaagtacttgacaaaatttcaccattaaagagaaatttgtgggagttcccatcgtggctcagtggaaacaaatccaactaggaaccatgaggttgtgggtttgatccctggcctcactcagtgggttaaggatccggtgttgccgtgagctgtggtgtaggttgcagacacggttctgatcctgcgttgctgtggctgtggctgtggtgtaggccagcagcaaacagctctgattagacccctagcctggaaacctccatatgccacaggtgcagccctaaaaagacaaaaaaagagaaaagacaaaaaaaaaaaaaaaaaaaaaaaaaaaaaaaaaaaaaaaaaaaagaacccccagaggtatttatttgtttttgccttttttcactgactgttctttgtttgtttgtttgagactgatctagaagactagagattacaagaaatatggatttggctcactctaagaaactgctttcattccaaggtttgggtctatccaaaagtggaatagaatcatatgaatactagtttatgagtatttagtgagaggaatttcaagctcaaataatgattcagcaagattaaattaaggagggaattttccttgtggctgagtgggttaaggacccaatgttgtctctgtgaggatgtaggttccatcctgggctttgctcattaggttaaggatctggcattgctgcagctcagacccagtgctgccctggttgtggcttaggccaaagctgcagctccaattcaatctctggcctgggaacctccatgtgctacaaggtgcggccttaaaaggaaaaaaaaaaaattaaatcaaggactcaagagtctttcattatttgtgttgtggaagctatatttgttttaaagtcttagttgtgtttagaaagcaagatgttcttcaactcaaatttgggagggaacttgtttcatacatttttaatggataagtggcaaaattttcatgctgaggtgatctatagtgttgtaatgcagaatatagtcagatcttgaacattttaggaagttggtgagggccaattgtgtatctgtgccatgctgataagaatgtcaagggatcacaagaattcgtgttatttgacagcagtcatctttaaaaggcatttgagaaagtccaatttcaaatgcatttcctttctttaaaagataaattgaagaaaataagtctttatttcccaagtaaattgaattgcctctcagtctgttaaaagaaactcttaccttgatgattgcgctcttaacctggcaaagattgtctttaaaatctgagctccatgtcttctgctttatttctggtgtgcctttgactccagattacagtaaatggaggactgagtatagggctaaaaagtagagagaatggatgcatattatctgtggtctccaatgtgatgaatgaagtaggcaaatactcaaaggaaagagaaagcatgctccaagaattatgggttccagaaggcaaagtcccagaattgtctccagggaaggacagggaggtctagaatcggctaagcccactgtaggcagaaaaaccaagaggcatgaatggcttccctttctcacttttcactctctggcttactcctatcatgaaggaaaatattggaatcatattctccctcaccgaaatgctatttttcagcccacaggaaacccaggctggttggagctgacatgccctgctctggtcgtgttgaagtaaaacatgcagacacgtggggctccgtctgtgattctgacttctctctgcatgcggccaacgtgctgtgcagggaactaaattgcggcgatgcgatttccctctcggtgggagatcactttggaaaaggaaatggactgacctgggctgaaaaattccagtgtgaggggagcgagacccaccttgcactctgcccaatagtacaacaccctgaagacacatgtatccacagcagggaagtcggcgtagtctgctcaagtaagagtttactgaaaataacactcttaaaatcttgttatgtttttattcataatgtgaatgagtagtagtggaaaataactaccagtttcctaagcttataacttcgtatagcatacattatacgaagttataagcctgcaggaattctaccgggtaggggaggcgcttttcccaaggcagtctggagcatgcgctttagcagccccgctgggcacttggcgctacacaagtggcctctggcctcgcacacattccacatccaccggtaggcgccaaccggctccgttctttggtggccccttcgcgccaccttctactcctcccctagtcaggaagttcccccccgccccgcagctcgcgtcgtgcaggacgtgacaaatggaagtagcacgtctcactagtctcgtgcagatggacagcaccgctgagcaatggaagcgggtaggcctttggggcagcggccaatagcagctttgctccttcgctttctgggctcagaggctgggaaggggtgggtccgggggcgggctcaggggcgggctcaggggcggggcgggcgcccgaaggtcctccggaggcccggcattctgcacgcttcaaaagcgcacgtctgccgcgctgttctcctcttcctcatctccgggcctttcgacctgcagccaccatggccatgattgaacaggatggcctgcatgcaggttctccagctgcctgggtggagagactgtttggctatgactgggcacagcagaccattggttgctctgatgcagcagtgttcagactgtcagcccagggcaggccagtcctgtttgtgaagacagacctcagtggggctctcaatgagctgcaggatgaggctgccagactctcctggctggcaacaactggggtcccctgtgcagctgtcctggatgtggtcacagaagctggaagggactggctcctgctgggtgaggtgcctgggcaggacctcctgtcctctcacctggctccagctgagaaagtgtcaatcatggctgatgccatgagaagactccacaccctggacccagccacctgcccctttgaccaccaggccaagcacaggattgagagggccagaaccaggatggaggctggcctggtggaccaggatgacctggatgaagaacaccagggcctggcccctgctgaactgtttgccaggctcaaggcatccatgccagatggtgaggacctggtggtgactcatggggatgcctgcctgcccaacatcatggtggaaaatggaaggttctctggcttcattgactgtggcaggctgggagtggctgacaggtaccaggacattgccctggcaaccagggacattgcagaagagctggggggagaatgggcagacaggttcctggtgctctatggcattgcagcccctgactcccagagaattgccttctacagactgctggatgagttcttctaaatcgattataatcagccataccacatttgtagaggttttacttgctttaaaaaacctcccacacctccccctgaacctgaaacataaaatgaatgcaatgttgttgttaaacttgtttattgcagcttataatggttacaaataaagcaatagcatcacaaatttcacaaataaagcatttttttcactgcattctagttgtggtttgtccaaactcatcaatgtggaaaataactaccagtttcctaagcttataacttcgtatagcatacattatacgaagttataagctagacaaaagtatcttaccccaatggtagccctgtacccaataaaagtaggtgttcagtttcatatcctatgaaataccctcttgatacttttactttgcatgaggatttagaagaaaaaagttttactataatccttaacttaggaaattcttttgaattggaaatgaaacacaaattgcttttcattgatatgccatatgattatatgaataaaacatgaaatcttcatattggattctagtatatacccaagtaaatattttttccctagaagagtgccaagtgtgttaaaaccttttggtttaataaagcagaaaaaaataaactctaaaaatcataattaaaaatgaaatgcttttatttatagcaattaactacaacatgtttagacttacatactattaaatataatatatttaagatcccctcatgataaatatgttcattattttgtaggctgttgatgcactaatatgtatgtagattactttgtgaattgcccttaataaaatttaaaactttaggctagtaaacctgtaacactcaacttagttctgaactatctcactattcttttgcaagaatttacttaggtaatgccaactaatttattccaaggccaaaaagatgacaatgtcttatatattataaaaactaataaaaaccattttaaaacctagtataaatttaaaggtacttgctcttctggttcatctcttcttttgtttacttctgctttcaaaaacttatttattgtgaccatattctttacttccatttattgttataatttataagatactatacttgcaagcaataaatgttatctttttagcttttaaatggtctcatttgaaaagaatatataattagtaagtcatagctactttaaataaaaacttattctttaagagattaaacacttctccaagtgatctgtttttctttaattaaaacgttattaactcccaaaatgatgttattgtttttttataatcttaaataccaataattaccaggtctattttgattttgatacaggataaaaactactattaattacttaagaatgtgttcttttttatatgtaccattttcatgatcaaagttggtgatatgactgaggttttgattattattaaacagatagttaatatgatatattcctcatttttccaaatgaaaggaaaaatgtcttatatggaggaaaagattggggcagggggattagtaaattattacttaaatatctgaataggaggatttttcaatgaaaggataaaggaagaatgattgtatcatctgaatctttccctccctttcctggagtttgtcctttcaacccagtatacctaccactcccttcatcacctactttcccattacagtccctatgtgttgggtggtaactattttgttttggtgttaatatccaagtttcccttaataacacctagtgaatggaggaaggatgagcatacctacccatcagacatatttagccaccatatttaatcaacaagcatgaagaaaggaagctagcctctccccttcctttcctcctgcctctctctctcttctctgtcctcgctccctttcttcccatcaatattttcagagcacctcttatgcgccaggcattgggatactcaaactggaggaaacaagaaaaaaaaaaaaaaaaggcgaagacctcagggaaatttatattgctgctatatttttttgagcctagtgtaaattaaaattccttaatgctgtgccttttaaaaacacaaataagcaaaatagtttatttcttcaacagttaaatccttagggtaggaaagtgattcaggatctattgctactattaactcttctttcattttcacacaggatacacacaaatccgcttggtgaatggcaagaccccatgtgaaggaagagtggagctcaacattcttgggtcctgggggtccctctgcaactctcactgggacatggaagatgcccatgttttatgccagcagcttaaatgtggagttgccctttctatcccgggaggagcaccttttgggaaaggaagtgagcaggtctggaggcacatgtttcactgcactgggactgagaagcacatgggagattgttccgtcactgctctgggcgcatcactctgttcttcagggcaagtggcctctgtaatctgctcaggtaagagaataagggcagccagtgatgagccactcatgacggtgccttaagagtgggtgtacctaggagttcccattgtggctcagtggtaacaaactcgactggtatccatgagggtatgggtttgatccctggccttgctcaatgggttaaggatccagcattgctgtgagctgtggtataggttgcagactctgctcaggtcccatgttgctgtgattgtggtgtaggctgactgctgcagcttcaatttgacccctagcccgggaatttccataggccacacgtgcagcactaaggaaggaaaaaaagaaaaaaaaaaaaaaagagtgggtgtgcctatagtgaagaacagatgtaaaagggaagtgaaagggattcccccattctgagggattgtgagaagtgtgccagaatattaacttcatttgacttgttacagggaaagtaaacttgactttcacggacctcctagttacctggtgcttactatatgtcttctcagagtacctgattcattcccagcctggttgacccatccccctatctctatggctatgtttatccagagcacatctatctaacactccagctgatcttcctgacacagctgtggcaaccctggatcctttaaccaactgtgccaggctggagatcaaacctaagcctctgcagcaacccaagctgctgcagtcagatttttaaccccctgtgccactgtgggtatctccgatattttgtatcttctgtgactgagtggtttgctgtttgcagggaaccagagtcagacactatccccgtgcaattcatcatcctcggacccatcaagctctattatttcagaagaaaatggtgttgcctgcataggtgagaatcagtgaccaacctatgaaaatgatctcaatcctctgaaatgcattttattcatgttttatttcctctttgcagggagtggtcaacttcgcctggtcgatggaggtggtcgttgtgctgggagagtagaggtctatcatgagggctcctggggcaccatctgtgatgacagctgggacctgaatgatgcccatgtggtgtgcaaacagctgagctgtggatgggccattaatgccactggttctgctcattttggggaaggaacagggcccatttggctggatgagataaactgtaatggaaaagaatctcatatttggcaatgccactcacatggttgggggcggcacaattgcaggcataaggaggatgcaggagtcatctgctcgg

SEQ ID NO: 119 - DNA, 4538 bp, Sus scrofa
  source 1..4538: mol_type = other DNA
tatagatgacaaggctttgtgtctgataggggccagcgaactcagtaaagagggaagatgagaaagataatggcaagaatttatccctgaagtgtagttttgacaaaccagtcacaaagaggtctaagaaattttggtcacaaagttgttttgaatcccaggcattttatttgcaatgattgcatatgttctggaaaggacatctgaacctaagaaatagttcatttgcattgtgttatattttactaaggtctgagaaataatcttgagatgagaatgaactctacttcttcagagtctggaaggaataaattatgaaaatgtattaatgcttctttaaaccatattgtatatttatctattactaaacaaaaagaagtagctctatttatttatttatttatttatttatttatgtcttttgtctctttagggccacacctgtggcatatggaggttcccaggctagaggtccaattggagatgtagcagccagcctatgccagagccaccgcaacacgggatctgagccacgtctgtgacttacaccacagctcacagcaacgcctgatcctcaacccactgagcgaggccagggatcgaacccatgtcctcatggatgctagttgggttcgttaactgctgagccatgatgggaactccaaattaattatttcttatatttgttcttcatatattcatttctatagaaagaaataaatacagattcagttaatgatggcaggtaaaagcttaacttattaatcaaaggagttaatccaggcacaaaaattcaattcatggctctctgttaaaatttaggtataggtttagcaggaagaaaaggttagtagatgcagactattacatttagaatggatggacaatgaagtcctactatacagcacagggaactatatccaatctcttgggatagaatatgatggaagacaaaatcagaacaagagagtatatatatatgtgtgtgtgtgtgtgtgtgtgtgtgtgtgtgtgtgtgtgtgtgtgactgggtcaccctgcggcacagcagaaattggcagaacattgtaaatcaactatactttaataggaaaaatacttttaagggctaaatttccaatattctaaccatgtacacagagtaaatgtcataaggatgccagtctgtgtagagattgatgtgttactagcagattcatgaaataaaggctgaggatgtagtccccaagtcacttctgagtggaagaatttctcctttgtcctggactcaaatattttaggataaaggaaaaaagaagatatttatagaagggacttgttttcaagtacttgacaaaatttcaccattaaagagaaatttgtgggagttcccatcgtggctcagtggaaacaaatccaactaggaaccatgaggttgtgggtttgatccctggcctcactcagtgggttaaggatccggtgttgccgtgagctgtggtgtaggttgcagacacggttctgatcctgcgttgctgtggctgtggctgtggtgtaggccagcagcaaacagctctgattagacccctagcctggaaacctccatatgccacaggtgcagccctaaaaagacaaaaaaagagaaaagacaaaaaaaaaaaaaaaaaaaaaaaaaaaaaaaaaaaaaaaaaaaagaacccccagaggtatttatttgtttttgccttttttcactgactgttctttgtttgtttgtttgagactgatctagaagactagagattacaagaaatatggatttggctcactctaagaaactgctttcattccaaggtttgggtctatccaaaagtggaatagaatcatatgaatactagtttatgagtatttagtgagaggaatttcaagctcaaataatgattcagcaagattaaattaaggagggaattttccttgtggctgagtgggttaaggacccaatgttgtctctgtgaggatgtaggttccatcctgggctttgctcattaggttaaggatctggcattgctgcagctcagacccagtgctgccctggttgtggcttaggccaaagctgcagctccaattcaatctctggcctgggaacctccatgtgctacaaggtgcggccttaaaaggaaaaaaaaaaaattaaatcaaggactcaagagtctttcattatttgtgttgtggaagctatatttgttttaaagtcttagttgtgtttagaaagcaagatgttcttcaactcaaatttgggagggaacttgtttcatacatttttaatggataagtggcaaaattttcatgctgaggtgatctatagtgttgtaatgcagaatatagtcagatcttgaacattttaggaagttggtgagggccaattgtgtatctgtgccatgctgataagaatgtcaagggatcacaagaattcgtgttatttgacagcagtcatctttaaaaggcatttgagaaagtccaatttcaaatgcatttcctttctttaaaagataaattgaagaaaataagtctttatttcccaagtaaattgaattgcctctcagtctgttaaaagaaactcttaccttgatgattgcgctcttaacctggcaaagattgtctttaaaatctgagctccatgtcttctgctttatttctggtgtgcctttgactccagattacagtaaatggaggactgagtatagggctaaaaagtagagagaatggatgcatattatctgtggtctccaatgtgatgaatgaagtaggcaaatactcaaaggaaagagaaagcatgctccaagaattatgggttccagaaggcaaagtcccagaattgtctccagggaaggacagggaggtctagaatcggctaagcccactgtaggcagaaaaaccaagaggcatgaatggcttccctttctcacttttcactctctggcttactcctatcatgaaggaaaatattggaatcatattctccctcaccgaaatgctatttttcagcccacaggaaacccagctcaacattcttgggtcctgggggtccctctgcaactctcactgggacatggaagatgcccatgttttatgccagcagcttaaatgtggagttgccctttctatcccgggaggagcaccttttgggaaaggaagtgagcaggtctggaggcacatgtttcactgcactgggactgagaagcacatgggagattgttccgtcactgctctgggcgcatcactctgttcttcagggcaagtggcctctgtaatctgctcaggtaagagaataagggcagccagtgatgagccactcatgacggtgccttaagagtgggtgtacctaggagttcccattgtggctcagtggtaacaaactcgactggtatccatgagggtatgggtttgatccctggccttgctcaatgggttaaggatccagcattgctgtgagctgtggtataggttgcagactctgctcaggtcccatgttgctgtgattgtggtgtaggctgactgctgcagcttcaatttgacccctagcccgggaatttccataggccacacgtgcagcactaaggaaggaaaaaaagaaaaaaaaaaaaaaagagtgggtgtgcctatagtgaagaacagatgtaaaagggaagtgaaagggattcccccattctgagggattgtgagaagtgtgccagaatattaacttcatttgacttgttacagggaaagtaaacttgactttcacggacctcctagttacctggtgcttactatatgtcttctcagagtacctgattcattcccagcctggttgacccatccccctatctctatggctatgtttatccagagcacatctatctaacactccagctgatcttcctgacacagctgtggcaaccctggatcctttaaccaactgtgccaggctggagatcaaacctaagcctctgcagcaacccaagctgctgcagtcagatttttaaccccctgtgccactgtgggtatctccgatattttgtatcttctgtgactgagtggtttgctgtttgcagggaaccagagtcagacactatccccgtgcaattcatcatcctcggacccatcaagctctattatttcagaagaaaatggtgttgcctgcataggtgagaatcagtgaccaacctatgaaaatgatctcaatcctctgaaatgcattttattcatgttttatttcctctttgcagggagtggtcaacttcgcctggtcgatggaggtggtcgttgtgctgggagagtagaggtctatcatgagggctcctggggcaccatctgtgatgacagctgggacctgaatgatgcccatgtggtgtgcaaacagctgagctgtggatgggccattaatgccactggttctgctcattttggggaaggaacagggcccatttggctggatgagataaactgtaatggaaaagaatctcatatttggcaatgccactcacatggttgggggcggcacaattgcaggcataaggaggatgcaggagtcatctgctcgg

SEQ ID NO: 120 - protein, 101 aa, Sus scrofa
PRLVGGDIPCSGRVEVQHGDTWGTVCDSDFSLEAASVLCRELQCGTVVSLLGGAHFGEGSGQIWAEEFQCEGHESHLSLCPVAPRPDGTCSHSRDVGVVCS

SEQ ID NO: 121 - protein, 100 aa, Homo sapiens
LRLVDGDSRCAGRVEIYHDGFWGTICDDGWDLSDAHVVCQKLGCGVAFNATVSAHFGEGSGPIWLDDLNCTGMESHLWQCPSRGWGQHDCRHKEDAGVIC